European Patent Specification EP 3 587 577 B1, published September 3, 2025. Title: Asymmetric siRNA Inhibiting Expression of Genes Directed to Male Type Depilation. Applicant: OLIX PHARMACEUTICALS, INC. The sequence listing filed with the application follows.

SEQUENCE LISTING (673 sequences)

SEQ ID NO: 1 - RNA, 16 nt, Artificial Sequence
  asiRNA
gcagauacuugagcca

SEQ ID NO: 2 - RNA, 16 nt, Artificial Sequence
  asiRNA
aagcagauacuugagc

SEQ ID NO: 3 - RNA, 16 nt, Artificial Sequence
  asiRNA
caaagcagauacuuga

SEQ ID NO: 4 - RNA, 16 nt, Artificial Sequence
  asiRNA
ugcaaagcagauacuu

SEQ ID NO: 5 - RNA, 16 nt, Artificial Sequence
  asiRNA
gugcaguguaugcuga

SEQ ID NO: 6 - RNA, 16 nt, Artificial Sequence
  asiRNA
uugugcaguguaugcu

SEQ ID NO: 7 - RNA, 16 nt, Artificial Sequence
  asiRNA
cauugugcaguguaug

SEQ ID NO: 8 - RNA, 16 nt, Artificial Sequence
  asiRNA
uuuuggcuugugguua

SEQ ID NO: 9 - RNA, 16 nt, Artificial Sequence
  asiRNA
cgggcauguugauaaa

SEQ ID NO: 10 - RNA, 16 nt, Artificial Sequence
  asiRNA
auauccuaaggaaucu

SEQ ID NO: 11 - RNA, 16 nt, Artificial Sequence
  asiRNA
aucucagaaaaccagg

SEQ ID NO: 12 - RNA, 16 nt, Artificial Sequence
  asiRNA
gaaucucagaaaacca

SEQ ID NO: 13 - RNA, 16 nt, Artificial Sequence
  asiRNA
aggaaucucagaaaac

SEQ ID NO: 14 - RNA, 16 nt, Artificial Sequence
  asiRNA
cuggauacaaaauacc

SEQ ID NO: 15 - RNA, 16 nt, Artificial Sequence
  asiRNA
uacuggauacaaaaua

SEQ ID NO: 16 - RNA, 16 nt, Artificial Sequence
  asiRNA
gauacuggauacaaaa

SEQ ID NO: 17 - RNA, 16 nt, Artificial Sequence
  asiRNA
gagauacuggauacaa

SEQ ID NO: 18 - RNA, 16 nt, Artificial Sequence
  asiRNA
aggagauacuggauac

SEQ ID NO: 19 - RNA, 16 nt, Artificial Sequence
  asiRNA
ccaggagauacuggau

SEQ ID NO: 20 - RNA, 16 nt, Artificial Sequence
  asiRNA
aauaccaaggggaggc

SEQ ID NO: 21 - RNA, 16 nt, Artificial Sequence
  asiRNA
aaaauaccaaggggag

SEQ ID NO: 22 - RNA, 16 nt, Artificial Sequence
  asiRNA
gaggcuuauuugaaua

SEQ ID NO: 23 - RNA, 16 nt, Artificial Sequence
  asiRNA
cagccaacuauuuugg

SEQ ID NO: 24 - RNA, 16 nt, Artificial Sequence
  asiRNA
ugcagccaacuauuuu

SEQ ID NO: 25 - RNA, 16 nt, Artificial Sequence
  asiRNA
acugcagccaacuauu

SEQ ID NO: 26 - RNA, 16 nt, Artificial Sequence
  asiRNA
uaacugcagccaacua

SEQ ID NO: 27 - RNA, 16 nt, Artificial Sequence
  asiRNA
cguaacugcagccaac

SEQ ID NO: 28 - RNA, 16 nt, Artificial Sequence
  asiRNA
auggagugguguggcu

SEQ ID NO: 29 - RNA, 16 nt, Artificial Sequence
  asiRNA
ucauggaguggugugg

SEQ ID NO: 30 - RNA, 16 nt, Artificial Sequence
  asiRNA
aaucauggaguggugu

SEQ ID NO: 31 - RNA, 16 nt, Artificial Sequence
  asiRNA
gaaaucauggaguggu

SEQ ID NO: 32 - RNA, 16 nt, Artificial Sequence
  asiRNA
gagaaaucauggagug

SEQ ID NO: 33 - RNA, 16 nt, Artificial Sequence
  asiRNA
cccuggccagcugguc

SEQ ID NO: 34 - RNA, 16 nt, Artificial Sequence
  asiRNA
uaugcccuggccagcu

SEQ ID NO: 35 - RNA, 16 nt, Artificial Sequence
  asiRNA
gcuaugcccuggccag

SEQ ID NO: 36 - RNA, 16 nt, Artificial Sequence
  asiRNA
ucaugagugguaccuc

SEQ ID NO: 37 - RNA, 16 nt, Artificial Sequence
  asiRNA
caucaugagugguacc

SEQ ID NO: 38 - RNA, 16 nt, Artificial Sequence
  asiRNA
uccggaaauuugaaga

SEQ ID NO: 39 - RNA, 16 nt, Artificial Sequence
  asiRNA
caguguaugcugauga

SEQ ID NO: 40 - RNA, 16 nt, Artificial Sequence
  asiRNA
gcauguugauaaacau

SEQ ID NO: 41 - RNA, 16 nt, Artificial Sequence
  asiRNA
guggcuaugcccuggc

SEQ ID NO: 42 - RNA, 16 nt, Artificial Sequence
  asiRNA
guguggcuaugcccug

SEQ ID NO: 43 - RNA, 16 nt, Artificial Sequence
  asiRNA
ugguguggcuaugccc

SEQ ID NO: 44 - RNA, 16 nt, Artificial Sequence
  asiRNA
agugguguggcuaugc

SEQ ID NO: 45 - RNA, 16 nt, Artificial Sequence
  asiRNA
ucuucacguuuuguuu

SEQ ID NO: 46 - RNA, 16 nt, Artificial Sequence
  asiRNA
gacuugagaacccuuu

SEQ ID NO: 47 - RNA, 16 nt, Artificial Sequence
  asiRNA
cuguuggcguguacaa

SEQ ID NO: 48 - RNA, 16 nt, Artificial Sequence
  asiRNA
uuauuugaauacguaa

SEQ ID NO: 49 - RNA, 16 nt, Artificial Sequence
  asiRNA
uuccaauggcgcuucu

SEQ ID NO: 50 - RNA, 16 nt, Artificial Sequence
  asiRNA
aaaggcaucuggacuu

SEQ ID NO: 51 - RNA, 16 nt, Artificial Sequence
  asiRNA
aucaaugugcucuggu

SEQ ID NO: 52 - RNA, 16 nt, Artificial Sequence
  asiRNA
gaucacuuucuguaac

SEQ ID NO: 53 - RNA, 16 nt, Artificial Sequence
  asiRNA
aucuuccuucuaauag

SEQ ID NO: 54 - RNA, 16 nt, Artificial Sequence
  asiRNA
ggcauugcuuugccuu

SEQ ID NO: 55 - RNA, 16 nt, Artificial Sequence
  asiRNA
uguacaauggcgauua

SEQ ID NO: 56 - RNA, 16 nt, Artificial Sequence
  asiRNA
cuucucuauggacuuu

SEQ ID NO: 57 - RNA, 16 nt, Artificial Sequence
  asiRNA
uuccaaggugaggcaa

SEQ ID NO: 58 - RNA, 16 nt, Artificial Sequence
  asiRNA
uccaaggugaggcaaa

SEQ ID NO: 59 - RNA, 16 nt, Artificial Sequence
  asiRNA
gguucauacggaguaa

SEQ ID NO: 60 - RNA, 16 nt, Artificial Sequence
  asiRNA
auaguagagauuguug

SEQ ID NO: 61 - RNA, 16 nt, Artificial Sequence
  asiRNA
uguugucugugaaauu

SEQ ID NO: 62 - RNA, 16 nt, Artificial Sequence
  asiRNA
uucaagcucuggguaa

SEQ ID NO: 63 - RNA, 16 nt, Artificial Sequence
  asiRNA
uaccuaauaaguaccu

SEQ ID NO: 64 - RNA, 16 nt, Artificial Sequence
  asiRNA
auuguugucugugaaa

SEQ ID NO: 65 - RNA, 16 nt, Artificial Sequence
  asiRNA
caaaagagcaucauga

SEQ ID NO: 66 - RNA, 16 nt, Artificial Sequence
  asiRNA
cuauggacuuuguaaa

SEQ ID NO: 67 - RNA, 16 nt, Artificial Sequence
  asiRNA
cugucuuugauggcau

SEQ ID NO: 68 - RNA, 16 nt, Artificial Sequence
  asiRNA
ucuaccuaauaaguac

SEQ ID NO: 69 - RNA, 16 nt, Artificial Sequence
  asiRNA
cuaaucuuccuucuaa

SEQ ID NO: 70 - RNA, 16 nt, Artificial Sequence
  asiRNA
cauuuucagaacaaua

SEQ ID NO: 71 - RNA, 16 nt, Artificial Sequence
  asiRNA
gaucucuucaagguca

SEQ ID NO: 72 - RNA, 16 nt, Artificial Sequence
  asiRNA
agauuguugucuguga

SEQ ID NO: 73 - RNA, 16 nt, Artificial Sequence
  asiRNA
agagauuguugucugu

SEQ ID NO: 74 - RNA, 16 nt, Artificial Sequence
  asiRNA
agacgaacucagugua

SEQ ID NO: 75 - RNA, 16 nt, Artificial Sequence
  asiRNA
uccuccuggccauguu

SEQ ID NO: 76 - RNA, 16 nt, Artificial Sequence
  asiRNA
cuuaauuuacccauuu

SEQ ID NO: 77 - RNA, 16 nt, Artificial Sequence
  asiRNA
ugaugcgaggaggaaa

SEQ ID NO: 78 - RNA, 16 nt, Artificial Sequence
  asiRNA
uguucuguaccuguaa

SEQ ID NO: 79 - RNA, 16 nt, Artificial Sequence
  asiRNA
ccuguaacggcuauuu

SEQ ID NO: 80 - RNA, 16 nt, Artificial Sequence
  asiRNA
ccauugugcaguguau

SEQ ID NO: 81 - RNA, 16 nt, Artificial Sequence
  asiRNA
aacauccauucagauc

SEQ ID NO: 82 - RNA, 16 nt, Artificial Sequence
  asiRNA
uauccaaaguucagaa

SEQ ID NO: 83 - RNA, 16 nt, Artificial Sequence
  asiRNA
accuaaauacgcugaa

SEQ ID NO: 84 - RNA, 16 nt, Artificial Sequence
  asiRNA
cgcugaaauggagguu

SEQ ID NO: 85 - RNA, 16 nt, Artificial Sequence
  asiRNA
aauggagguugaauau

SEQ ID NO: 86 - RNA, 16 nt, Artificial Sequence
  asiRNA
auauccuacuguguaa

SEQ ID NO: 87 - RNA, 16 nt, Artificial Sequence
  asiRNA
uaugagacuagacuuu

SEQ ID NO: 88 - RNA, 16 nt, Artificial Sequence
  asiRNA
aaugucacaaucccuu

SEQ ID NO: 89 - RNA, 16 nt, Artificial Sequence
  asiRNA
ggucaacugcaguguu

SEQ ID NO: 90 - RNA, 16 nt, Artificial Sequence
  asiRNA
gccauugugcagucau

SEQ ID NO: 91 - RNA, 16 nt, Artificial Sequence
  asiRNA
uguaaguggagaacuu

SEQ ID NO: 92 - RNA, 16 nt, Artificial Sequence
  asiRNA
cucugccugugugagu

SEQ ID NO: 93 - RNA, 16 nt, Artificial Sequence
  asiRNA
accgugagccaucaau

SEQ ID NO: 94 - RNA, 16 nt, Artificial Sequence
  asiRNA
gguuucucucugucuu

SEQ ID NO: 95 - RNA, 16 nt, Artificial Sequence
  asiRNA
uagucuagaccuaguu

SEQ ID NO: 96 - RNA, 16 nt, Artificial Sequence
  asiRNA
uaguguaaagaaugau

SEQ ID NO: 97 - RNA, 16 nt, Artificial Sequence
  asiRNA
cuguaccuguuaucaa

SEQ ID NO: 98 - RNA, 16 nt, Artificial Sequence
  asiRNA
gaaugcuucaugacuu

SEQ ID NO: 99 - RNA, 16 nt, Artificial Sequence
  asiRNA
ugccuuaucaucucau

SEQ ID NO: 100 - RNA, 16 nt, Artificial Sequence
  asiRNA
caucucaucuggaguu

SEQ ID NO: 101 - RNA, 21 nt, Artificial Sequence
  asiRNA
uggcucaaguaucugcuuugc

SEQ ID NO: 102 - RNA, 21 nt, Artificial Sequence
  asiRNA
gcucaaguaucugcuuugcaa

SEQ ID NO: 103 - RNA, 21 nt, Artificial Sequence
  asiRNA
ucaaguaucugcuuugcaaau

SEQ ID NO: 104 - RNA, 21 nt, Artificial Sequence
  asiRNA
aaguaucugcuuugcaaauag

SEQ ID NO: 105 - RNA, 21 nt, Artificial Sequence
  asiRNA
ucagcauacacugcacaaugg

SEQ ID NO: 106 - RNA, 21 nt, Artificial Sequence
  asiRNA
agcauacacugcacaauggcu

SEQ ID NO: 107 - RNA, 21 nt, Artificial Sequence
  asiRNA
cauacacugcacaauggcuca

SEQ ID NO: 108 - RNA, 21 nt, Artificial Sequence
  asiRNA
uaaccacaagccaaaaccuau

SEQ ID NO: 109 - RNA, 21 nt, Artificial Sequence
  asiRNA
uuuaucaacaugcccguuaac

SEQ ID NO: 110 - RNA, 21 nt, Artificial Sequence
  asiRNA
agauuccuuaggauaugaucu

SEQ ID NO: 111 - RNA, 21 nt, Artificial Sequence
  asiRNA
ccugguuuucugagauuccuu

SEQ ID NO: 112 - RNA, 21 nt, Artificial Sequence
  asiRNA
ugguuuucugagauuccuuag

SEQ ID NO: 113 - RNA, 21 nt, Artificial Sequence
  asiRNA
guuuucugagauuccuuagga

SEQ ID NO: 114 - RNA, 21 nt, Artificial Sequence
  asiRNA
gguauuuuguauccaguaucu

SEQ ID NO: 115 - RNA, 21 nt, Artificial Sequence
  asiRNA
uauuuuguauccaguaucucc

SEQ ID NO: 116 - RNA, 21 nt, Artificial Sequence
  asiRNA
uuuuguauccaguaucuccug

SEQ ID NO: 117 - RNA, 21 nt, Artificial Sequence
  asiRNA
uuguauccaguaucuccuggu

SEQ ID NO: 118 - RNA, 21 nt, Artificial Sequence
  asiRNA
guauccaguaucuccugguuu

SEQ ID NO: 119 - RNA, 21 nt, Artificial Sequence
  asiRNA
auccaguaucuccugguuuuc

SEQ ID NO: 120 - RNA, 21 nt, Artificial Sequence
  asiRNA
gccuccccuugguauuuugua

SEQ ID NO: 121 - RNA, 21 nt, Artificial Sequence
  asiRNA
cuccccuugguauuuuguauc

SEQ ID NO: 122 - RNA, 21 nt, Artificial Sequence
  asiRNA
uauucaaauaagccuccccuu

SEQ ID NO: 123 - RNA, 21 nt, Artificial Sequence
  asiRNA
ccaaaauaguuggcugcaguu

SEQ ID NO: 124 - RNA, 21 nt, Artificial Sequence
  asiRNA
aaaauaguuggcugcaguuac

SEQ ID NO: 125 - RNA, 21 nt, Artificial Sequence
  asiRNA
aauaguuggcugcaguuacgu

SEQ ID NO: 126 - RNA, 21 nt, Artificial Sequence
  asiRNA
uaguuggcugcaguuacguau

SEQ ID NO: 127 - RNA, 21 nt, Artificial Sequence
  asiRNA
guuggcugcaguuacguauuc

SEQ ID NO: 128 - RNA, 21 nt, Artificial Sequence
  asiRNA
agccacaccacuccaugauuu

SEQ ID NO: 129 - RNA, 21 nt, Artificial Sequence
  asiRNA
ccacaccacuccaugauuucu

SEQ ID NO: 130 - RNA, 21 nt, Artificial Sequence
  asiRNA
acaccacuccaugauuucucc

SEQ ID NO: 131 - RNA, 21 nt, Artificial Sequence
  asiRNA
accacuccaugauuucuccaa

SEQ ID NO: 132 - RNA, 21 nt, Artificial Sequence
  asiRNA
cacuccaugauuucuccaaaa

SEQ ID NO: 133 - RNA, 21 nt, Artificial Sequence
  asiRNA
gaccagcuggccagggcauag

SEQ ID NO: 134 - RNA, 21 nt, Artificial Sequence
  asiRNA
agcuggccagggcauagccac

SEQ ID NO: 135 - RNA, 21 nt, Artificial Sequence
  asiRNA
cuggccagggcauagccacac

SEQ ID NO: 136 - RNA, 21 nt, Artificial Sequence
  asiRNA
gagguaccacucaugaugcuc

SEQ ID NO: 137 - RNA, 21 nt, Artificial Sequence
  asiRNA
gguaccacucaugaugcucuu

SEQ ID NO: 138 - RNA, 21 nt, Artificial Sequence
  asiRNA
ucuucaaauuuccggagguac

SEQ ID NO: 139 - RNA, 21 nt, Artificial Sequence
  asiRNA
ucaucagcauacacugcacaa

SEQ ID NO: 140 - RNA, 21 nt, Artificial Sequence
  asiRNA
auguuuaucaacaugcccguu

SEQ ID NO: 141 - RNA, 21 nt, Artificial Sequence
  asiRNA
gccagggcauagccacaccac

SEQ ID NO: 142 - RNA, 21 nt, Artificial Sequence
  asiRNA
cagggcauagccacaccacuc

SEQ ID NO: 143 - RNA, 21 nt, Artificial Sequence
  asiRNA
gggcauagccacaccacucca

SEQ ID NO: 144 - RNA, 21 nt, Artificial Sequence
  asiRNA
gcauagccacaccacuccaug

SEQ ID NO: 145 - RNA, 21 nt, Artificial Sequence
  asiRNA
aaacaaaacgugaagaaagca

SEQ ID NO: 146 - RNA, 21 nt, Artificial Sequence
  asiRNA
aaaggguucucaagucaggcu

SEQ ID NO: 147 - RNA, 21 nt, Artificial Sequence
  asiRNA
uuguacacgccaacaguggca

SEQ ID NO: 148 - RNA, 21 nt, Artificial Sequence
  asiRNA
uuacguauucaaauaagccuc

SEQ ID NO: 149 - RNA, 21 nt, Artificial Sequence
  asiRNA
agaagcgccauuggaaagcuu

SEQ ID NO: 150 - RNA, 21 nt, Artificial Sequence
  asiRNA
aaguccagaugccuuugccuc

SEQ ID NO: 151 - RNA, 21 nt, Artificial Sequence
  asiRNA
accagagcacauugauggcuc

SEQ ID NO: 152 - RNA, 21 nt, Artificial Sequence
  asiRNA
guuacagaaagugaucauucu

SEQ ID NO: 153 - RNA, 21 nt, Artificial Sequence
  asiRNA
cuauuagaaggaagauuagcu

SEQ ID NO: 154 - RNA, 21 nt, Artificial Sequence
  asiRNA
aaggcaaagcaaugccagaug

SEQ ID NO: 155 - RNA, 21 nt, Artificial Sequence
  asiRNA
uaaucgccauuguacacgcca

SEQ ID NO: 156 - RNA, 21 nt, Artificial Sequence
  asiRNA
aaaguccauagagaagcgcca

SEQ ID NO: 157 - RNA, 21 nt, Artificial Sequence
  asiRNA
uugccucaccuuggaagggcc

SEQ ID NO: 158 - RNA, 21 nt, Artificial Sequence
  asiRNA
uuugccucaccuuggaagggc

SEQ ID NO: 159 - RNA, 21 nt, Artificial Sequence
  asiRNA
uuacuccguaugaaccaccac

SEQ ID NO: 160 - RNA, 21 nt, Artificial Sequence
  asiRNA
caacaaucucuacuauaucca

SEQ ID NO: 161 - RNA, 21 nt, Artificial Sequence
  asiRNA
aauuucacagacaacaaucuc

SEQ ID NO: 162 - RNA, 21 nt, Artificial Sequence
  asiRNA
uuacccagagcuugaaauucu

SEQ ID NO: 163 - RNA, 21 nt, Artificial Sequence
  asiRNA
agguacuuauuagguagauug

SEQ ID NO: 164 - RNA, 21 nt, Artificial Sequence
  asiRNA
uuucacagacaacaaucucua

SEQ ID NO: 165 - RNA, 21 nt, Artificial Sequence
  asiRNA
ucaugaugcucuuuugcucua

SEQ ID NO: 166 - RNA, 21 nt, Artificial Sequence
  asiRNA
uuuacaaaguccauagagaag

SEQ ID NO: 167 - RNA, 21 nt, Artificial Sequence
  asiRNA
augccaucaaagacaguugua

SEQ ID NO: 168 - RNA, 21 nt, Artificial Sequence
  asiRNA
guacuuauuagguagauugca

SEQ ID NO: 169 - RNA, 21 nt, Artificial Sequence
  asiRNA
uuagaaggaagauuagcuaug

SEQ ID NO: 170 - RNA, 21 nt, Artificial Sequence
  asiRNA
uauuguucugaaaaugccauc

SEQ ID NO: 171 - RNA, 21 nt, Artificial Sequence
  asiRNA
ugaccuugaagagaucacugu

SEQ ID NO: 172 - RNA, 21 nt, Artificial Sequence
  asiRNA
ucacagacaacaaucucuacu

SEQ ID NO: 173 - RNA, 21 nt, Artificial Sequence
  asiRNA
acagacaacaaucucuacuau

SEQ ID NO: 174 - RNA, 21 nt, Artificial Sequence
  asiRNA
uacacugaguucgucugacga

SEQ ID NO: 175 - RNA, 21 nt, Artificial Sequence
  asiRNA
aacauggccaggaggaugcag

SEQ ID NO: 176 - RNA, 21 nt, Artificial Sequence
  asiRNA
aaauggguaaauuaagcaccg

SEQ ID NO: 177 - RNA, 21 nt, Artificial Sequence
  asiRNA
uuuccuccucgcaucagaaau

SEQ ID NO: 178 - RNA, 21 nt, Artificial Sequence
  asiRNA
uuacagguacagaacauaauc

SEQ ID NO: 179 - RNA, 21 nt, Artificial Sequence
  asiRNA
aaauagccguuacagguacag

SEQ ID NO: 180 - RNA, 21 nt, Artificial Sequence
  asiRNA
auacacugcacaauggcucaa

SEQ ID NO: 181 - RNA, 21 nt, Artificial Sequence
  asiRNA
gaucugaauggauguuuauca

SEQ ID NO: 182 - RNA, 21 nt, Artificial Sequence
  asiRNA
uucugaacuuuggauacucuu

SEQ ID NO: 183 - RNA, 21 nt, Artificial Sequence
  asiRNA
uucagcguauuuagguacuua

SEQ ID NO: 184 - RNA, 21 nt, Artificial Sequence
  asiRNA
aaccuccauuucagcguauuu

SEQ ID NO: 185 - RNA, 21 nt, Artificial Sequence
  asiRNA
auauucaaccuccauuucagc

SEQ ID NO: 186 - RNA, 21 nt, Artificial Sequence
  asiRNA
uuacacaguaggauauucaac

SEQ ID NO: 187 - RNA, 21 nt, Artificial Sequence
  asiRNA
aaagucuagucucauacacac

SEQ ID NO: 188 - RNA, 21 nt, Artificial Sequence
  asiRNA
aagggauugugacauuuauug

SEQ ID NO: 189 - RNA, 21 nt, Artificial Sequence
  asiRNA
aacacugcaguugaccuugaa

SEQ ID NO: 190 - RNA, 21 nt, Artificial Sequence
  asiRNA
augacugcacaauggcuaccc

SEQ ID NO: 191 - RNA, 21 nt, Artificial Sequence
  asiRNA
aaguucuccacuuacacacag

SEQ ID NO: 192 - RNA, 21 nt, Artificial Sequence
  asiRNA
acucacacaggcagagcagcu

SEQ ID NO: 193 - RNA, 21 nt, Artificial Sequence
  asiRNA
auugauggcucacggugagug

SEQ ID NO: 194 - RNA, 21 nt, Artificial Sequence
  asiRNA
aagacagagagaaaccauguc

SEQ ID NO: 195 - RNA, 21 nt, Artificial Sequence
  asiRNA
aacuaggucuagacuagaaga

SEQ ID NO: 196 - RNA, 21 nt, Artificial Sequence
  asiRNA
aucauucuuuacacuacaagg

SEQ ID NO: 197 - RNA, 21 nt, Artificial Sequence
  asiRNA
uugauaacagguacaggcuau

SEQ ID NO: 198 - RNA, 21 nt, Artificial Sequence
  asiRNA
aagucaugaagcauucaacag

SEQ ID NO: 199 - RNA, 21 nt, Artificial Sequence
  asiRNA
augagaugauaaggcaaagca

SEQ ID NO: 200 - RNA, 21 nt, Artificial Sequence
  asiRNA
aacuccagaugagaugauaag

SEQ ID NO: 201 - RNA, 16 nt, Artificial Sequence
  asiRNA
guuccugcaggagcug

SEQ ID NO: 202 - RNA, 16 nt, Artificial Sequence
  asiRNA
uuccugcaggagcugc

SEQ ID NO: 203 - RNA, 16 nt, Artificial Sequence
  asiRNA
uccugcaggagcugcc

SEQ ID NO: 204 - RNA, 16 nt, Artificial Sequence
  asiRNA
ccugcaggagcugccu

SEQ ID NO: 205 - RNA, 16 nt, Artificial Sequence
  asiRNA
cugcaggagcugccuu

SEQ ID NO: 206 - RNA, 16 nt, Artificial Sequence
  asiRNA
ugcaggagcugccuuc

SEQ ID NO: 207 - RNA, 16 nt, Artificial Sequence
  asiRNA
gcaggagcugccuucc

SEQ ID NO: 208 - RNA, 16 nt, Artificial Sequence
  asiRNA
caggagcugccuuccu

SEQ ID NO: 209 - RNA, 16 nt, Artificial Sequence
  asiRNA
aggagcugccuuccuu

SEQ ID NO: 210 - RNA, 16 nt, Artificial Sequence
  asiRNA
acuuccacaggacauu

SEQ ID NO: 211 - RNA, 16 nt, Artificial Sequence
  asiRNA
cuuccacaggacauuu

SEQ ID NO: 212 - RNA, 16 nt, Artificial Sequence
  asiRNA
agguggcuuguuuacg

SEQ ID NO: 213 - RNA, 16 nt, Artificial Sequence
  asiRNA
gguggcuuguuuacgu

SEQ ID NO: 214 - RNA, 16 nt, Artificial Sequence
  asiRNA
guggcuuguuuacgua

SEQ ID NO: 215 - RNA, 16 nt, Artificial Sequence
  asiRNA
uggcuuguuuacguau

SEQ ID NO: 216 - RNA, 16 nt, Artificial Sequence
  asiRNA
ggcuuguuuacguaug

SEQ ID NO: 217 - RNA, 16 nt, Artificial Sequence
  asiRNA
gcuuguuuacguaugu

SEQ ID NO: 218 - RNA, 16 nt, Artificial Sequence
  asiRNA
cuaccucaagauguuu

SEQ ID NO: 219 - RNA, 16 nt, Artificial Sequence
  asiRNA
gguuccugcaggagcu

SEQ ID NO: 220 - RNA, 16 nt, Artificial Sequence
  asiRNA
uacuuccacaggacau

SEQ ID NO: 221 - RNA, 16 nt, Artificial Sequence
  asiRNA
agacauacgguuuagc

SEQ ID NO: 222 - RNA, 16 nt, Artificial Sequence
  asiRNA
cagacauacgguuuag

SEQ ID NO: 223 - RNA, 16 nt, Artificial Sequence
  asiRNA
acagacauacgguuua

SEQ ID NO: 224 - RNA, 16 nt, Artificial Sequence
  asiRNA
cacagacauacgguuu

SEQ ID NO: 225 - RNA, 16 nt, Artificial Sequence
  asiRNA
ggauuccacaaggugg

SEQ ID NO: 226 - RNA, 16 nt, Artificial Sequence
  asiRNA
gauuccacaagguggc

SEQ ID NO: 227 - RNA, 16 nt, Artificial Sequence
  asiRNA
auuccacaagguggcu

SEQ ID NO: 228 - RNA, 16 nt, Artificial Sequence
  asiRNA
uuccacaagguggcuu

SEQ ID NO: 229 - RNA, 16 nt, Artificial Sequence
  asiRNA
uccacaagguggcuug

SEQ ID NO: 230 - RNA, 16 nt, Artificial Sequence
  asiRNA
ccacaagguggcuugu

SEQ ID NO: 231 - RNA, 16 nt, Artificial Sequence
  asiRNA
cacaagguggcuuguu

SEQ ID NO: 232 - RNA, 16 nt, Artificial Sequence
  asiRNA
acaagguggcuuguuu

SEQ ID NO: 233 - RNA, 16 nt, Artificial Sequence
  asiRNA
caagguggcuuguuua

SEQ ID NO: 234 - RNA, 16 nt, Artificial Sequence
  asiRNA
aagguggcuuguuuac

SEQ ID NO: 235 - RNA, 16 nt, Artificial Sequence
  asiRNA
cuggagccaauuuccu

SEQ ID NO: 236 - RNA, 16 nt, Artificial Sequence
  asiRNA
ucuggagccaauuucc

SEQ ID NO: 237 - RNA, 16 nt, Artificial Sequence
  asiRNA
uucuggagccaauuuc

SEQ ID NO: 238 - RNA, 16 nt, Artificial Sequence
  asiRNA
uuucuggagccaauuu

SEQ ID NO: 239 - RNA, 16 nt, Artificial Sequence
  asiRNA
guuucuggagccaauu

SEQ ID NO: 240 - RNA, 16 nt, Artificial Sequence
  asiRNA
uguuucuggagccaau

SEQ ID NO: 241 - RNA, 16 nt, Artificial Sequence
  asiRNA
auguuucuggagccaa

SEQ ID NO: 242 - RNA, 16 nt, Artificial Sequence
  asiRNA
uauguuucuggagcca

SEQ ID NO: 243 - RNA, 16 nt, Artificial Sequence
  asiRNA
guauguuucuggagcc

SEQ ID NO: 244 - RNA, 16 nt, Artificial Sequence
  asiRNA
gcuccagaaacauacg

SEQ ID NO: 245 - RNA, 16 nt, Artificial Sequence
  asiRNA
cauagguucuaccuca

SEQ ID NO: 246 - RNA, 16 nt, Artificial Sequence
  asiRNA
auagguucuaccucaa

SEQ ID NO: 247 - RNA, 16 nt, Artificial Sequence
  asiRNA
uagguucuaccucaag

SEQ ID NO: 248 - RNA, 16 nt, Artificial Sequence
  asiRNA
agguucuaccucaaga

SEQ ID NO: 249 - RNA, 16 nt, Artificial Sequence
  asiRNA
gguucuaccucaagau

SEQ ID NO: 250 - RNA, 16 nt, Artificial Sequence
  asiRNA
guucuaccucaagaug

SEQ ID NO: 251 - RNA, 16 nt, Artificial Sequence
  asiRNA
uucuaccucaagaugu

SEQ ID NO: 252 - RNA, 16 nt, Artificial Sequence
  asiRNA
ucuaccucaagauguu

SEQ ID NO: 253 - RNA, 16 nt, Artificial Sequence
  asiRNA
caaaucucggaaagcc

SEQ ID NO: 254 - RNA, 16 nt, Artificial Sequence
  asiRNA
aaaucucggaaagccc

SEQ ID NO: 255 - RNA, 16 nt, Artificial Sequence
  asiRNA
aaucucggaaagcccu

SEQ ID NO: 256 - RNA, 16 nt, Artificial Sequence
  asiRNA
gcccuuauuccauuca

SEQ ID NO: 257 - RNA, 16 nt, Artificial Sequence
  asiRNA
cccuuauuccauucau

SEQ ID NO: 258 - RNA, 16 nt, Artificial Sequence
  asiRNA
ccuuauuccauucauc

SEQ ID NO: 259 - RNA, 16 nt, Artificial Sequence
  asiRNA
cuuauuccauucaucu

SEQ ID NO: 260 - RNA, 16 nt, Artificial Sequence
  asiRNA
uuauuccauucaucuu

SEQ ID NO: 261 - RNA, 16 nt, Artificial Sequence
  asiRNA
uauuccauucaucuuu

SEQ ID NO: 262 - RNA, 16 nt, Artificial Sequence
  asiRNA
auuccauucaucuuuu

SEQ ID NO: 263 - RNA, 16 nt, Artificial Sequence
  asiRNA
uuccauucaucuuuua

SEQ ID NO: 264 - RNA, 16 nt, Artificial Sequence
  asiRNA
uccauucaucuuuuaa

SEQ ID NO: 265 - RNA, 16 nt, Artificial Sequence
  asiRNA
ucucacuuuguuuccu

SEQ ID NO: 266 - RNA, 16 nt, Artificial Sequence
  asiRNA
uucucacuuuguuucc

SEQ ID NO: 267 - RNA, 16 nt, Artificial Sequence
  asiRNA
uuucucacuuuguuuc

SEQ ID NO: 268 - RNA, 16 nt, Artificial Sequence
  asiRNA
uuuucucacuuuguuu

SEQ ID NO: 269 - RNA, 16 nt, Artificial Sequence
  asiRNA
uuuuucucacuuuguu

SEQ ID NO: 270 - RNA, 16 nt, Artificial Sequence
  asiRNA
auuuuucucacuuugu

SEQ ID NO: 271 - RNA, 16 nt, Artificial Sequence
  asiRNA
uggcaggcagcgccac

SEQ ID NO: 272 - RNA, 16 nt, Artificial Sequence
  asiRNA
cuggcaggcagcgcca

SEQ ID NO: 273 - RNA, 16 nt, Artificial Sequence
  asiRNA
ggcaggcagcgccacu

SEQ ID NO: 274 - RNA, 16 nt, Artificial Sequence
  asiRNA
ugccagcccgcgccgc

SEQ ID NO: 275 - RNA, 16 nt, Artificial Sequence
  asiRNA
uuacuuccacaggaca

SEQ ID NO: 276 - RNA, 16 nt, Artificial Sequence
  asiRNA
guggaaguaauguagg

SEQ ID NO: 277 - RNA, 16 nt, Artificial Sequence
  asiRNA
cccugaugggugguac

SEQ ID NO: 278 - RNA, 16 nt, Artificial Sequence
  asiRNA
ccugaugggugguaca

SEQ ID NO: 279 - RNA, 16 nt, Artificial Sequence
  asiRNA
cugaugggugguacac

SEQ ID NO: 280 - RNA, 16 nt, Artificial Sequence
  asiRNA
ugaugggugguacaca

SEQ ID NO: 281 - RNA, 16 nt, Artificial Sequence
  asiRNA
gaugggugguacacag

SEQ ID NO: 282 - RNA, 16 nt, Artificial Sequence
  asiRNA
augggugguacacaga

SEQ ID NO: 283 - RNA, 16 nt, Artificial Sequence
  asiRNA
ugggugguacacagac

SEQ ID NO: 284 - RNA, 16 nt, Artificial Sequence
  asiRNA
gggugguacacagaca

SEQ ID NO: 285 - RNA, 16 nt, Artificial Sequence
  asiRNA
ggugguacacagacau

SEQ ID NO: 286 - RNA, 16 nt, Artificial Sequence
  asiRNA
gacauacgguuuagcu

SEQ ID NO: 287 - RNA, 16 nt, Artificial Sequence
  asiRNA
cuugggugucuucuua

SEQ ID NO: 288 - RNA, 16 nt, Artificial Sequence
  asiRNA
gcuugggugucuucuu

SEQ ID NO: 289 - RNA, 16 nt, Artificial Sequence
  asiRNA
agcuugggugucuucu

SEQ ID NO: 290 - RNA, 16 nt, Artificial Sequence
  asiRNA
uagcuugggugucuuc

SEQ ID NO: 291 - RNA, 16 nt, Artificial Sequence
  asiRNA
gccagcucaggaagcc

SEQ ID NO: 292 - RNA, 16 nt, Artificial Sequence
  asiRNA
cgccagcucaggaagc

SEQ ID NO: 293 - RNA, 16 nt, Artificial Sequence
  asiRNA
gcgccagcucaggaag

SEQ ID NO: 294 - RNA, 16 nt, Artificial Sequence
  asiRNA
uggagccaauuuccuc

SEQ ID NO: 295 - RNA, 16 nt, Artificial Sequence
  asiRNA
cucacuuuguuuccuu

SEQ ID NO: 296 - RNA, 16 nt, Artificial Sequence
  asiRNA
cauuuuucucacuuug

SEQ ID NO: 297 - RNA, 16 nt, Artificial Sequence
  asiRNA
ccauagguucuaccuc

SEQ ID NO: 298 - RNA, 16 nt, Artificial Sequence
  asiRNA
accauagguucuaccu

SEQ ID NO: 299 - RNA, 16 nt, Artificial Sequence
  asiRNA
caccauagguucuacc

SEQ ID NO: 300 - RNA, 16 nt, Artificial Sequence
  asiRNA
ccaccauagguucuac

SEQ ID NO: 301 - RNA, 16 nt, Artificial Sequence
  asiRNA
accaccauagguucua

SEQ ID NO: 302 - RNA, 16 nt, Artificial Sequence
  asiRNA
caccaccauagguucu

SEQ ID NO: 303 - RNA, 16 nt, Artificial Sequence
  asiRNA
ggacuaccccaaaucu

SEQ ID NO: 304 - RNA, 16 nt, Artificial Sequence
  asiRNA
aggacuaccccaaauc

SEQ ID NO: 305 - RNA, 16 nt, Artificial Sequence
  asiRNA
gaggacuaccccaaau

SEQ ID NO: 306 - RNA, 16 nt, Artificial Sequence
  asiRNA
ugaggacuaccccaaa

SEQ ID NO: 307 - RNA, 16 nt, Artificial Sequence
  asiRNA
uugaggacuaccccaa

SEQ ID NO: 308 - RNA, 16 nt, Artificial Sequence
  asiRNA
uuugaggacuacccca

SEQ ID NO: 309 - RNA, 16 nt, Artificial Sequence
  asiRNA
ccaaaucucggaaagc

SEQ ID NO: 310 - RNA, 16 nt, Artificial Sequence
  asiRNA
agcccuuauuccauuc

SEQ ID NO: 311 - RNA, 16 nt, Artificial Sequence
  asiRNA
aagcccuuauuccauu

SEQ ID NO: 312 - RNA, 16 nt, Artificial Sequence
  asiRNA
ggcuaugcccuggcca

SEQ ID NO: 313 - RNA, 21 nt, Artificial Sequence
  asiRNA
cagcuccugcaggaaccaggc

SEQ ID NO: 314 - RNA, 21 nt, Artificial Sequence
  asiRNA
gcagcuccugcaggaaccagg

SEQ ID NO: 315 - RNA, 21 nt, Artificial Sequence
  asiRNA
ggcagcuccugcaggaaccag

SEQ ID NO: 316 - RNA, 21 nt, Artificial Sequence
  asiRNA
aggcagcuccugcaggaacca

SEQ ID NO: 317 - RNA, 21 nt, Artificial Sequence
  asiRNA
aaggcagcuccugcaggaacc

SEQ ID NO: 318 - RNA, 21 nt, Artificial Sequence
  asiRNA
gaaggcagcuccugcaggaac

SEQ ID NO: 319 - RNA, 21 nt, Artificial Sequence
  asiRNA
ggaaggcagcuccugcaggaa

SEQ ID NO: 320 - RNA, 21 nt, Artificial Sequence
  asiRNA
aggaaggcagcuccugcagga

SEQ ID NO: 321 - RNA, 21 nt, Artificial Sequence
  asiRNA
aaggaaggcagcuccugcagg

SEQ ID NO: 322 - RNA, 21 nt, Artificial Sequence
  asiRNA
aauguccuguggaaguaaugu

SEQ ID NO: 323 - RNA, 21 nt, Artificial Sequence
  asiRNA
aaauguccuguggaaguaaug

SEQ ID NO: 324 - RNA, 21 nt, Artificial Sequence
  asiRNA
cguaaacaagccaccuugugg

SEQ ID NO: 325 - RNA, 21 nt, Artificial Sequence
  asiRNA
acguaaacaagccaccuugug

SEQ ID NO: 326 - RNA, 21 nt, Artificial Sequence
  asiRNA
uacguaaacaagccaccuugu

SEQ ID NO: 327 - RNA, 21 nt, Artificial Sequence
  asiRNA
auacguaaacaagccaccuug

SEQ ID NO: 328 - RNA, 21 nt, Artificial Sequence
  asiRNA
cauacguaaacaagccaccuu

SEQ ID NO: 329 - RNA, 21 nt, Artificial Sequence
  asiRNA
acauacguaaacaagccaccu

SEQ ID NO: 330 - RNA, 21 nt, Artificial Sequence
  asiRNA
aaacaucuugagguagaaccu

SEQ ID NO: 331 - RNA, 21 nt, Artificial Sequence
  asiRNA
agcuccugcaggaaccaggcg

SEQ ID NO: 332 - RNA, 21 nt, Artificial Sequence
  asiRNA
auguccuguggaaguaaugua

SEQ ID NO: 333 - RNA, 21 nt, Artificial Sequence
  asiRNA
gcuaaaccguaugucugugua

SEQ ID NO: 334 - RNA, 21 nt, Artificial Sequence
  asiRNA
cuaaaccguaugucuguguac

SEQ ID NO: 335 - RNA, 21 nt, Artificial Sequence
  asiRNA
uaaaccguaugucuguguacc

SEQ ID NO: 336 - RNA, 21 nt, Artificial Sequence
  asiRNA
aaaccguaugucuguguacca

SEQ ID NO: 337 - RNA, 21 nt, Artificial Sequence
  asiRNA
ccaccuuguggaauccuguag

SEQ ID NO: 338 - RNA, 21 nt, Artificial Sequence
  asiRNA
gccaccuuguggaauccugua

SEQ ID NO: 339 - RNA, 21 nt, Artificial Sequence
  asiRNA
agccaccuuguggaauccugu

SEQ ID NO: 340 - RNA, 21 nt, Artificial Sequence
  asiRNA
aagccaccuuguggaauccug

SEQ ID NO: 341 - RNA, 21 nt, Artificial Sequence
  asiRNA
caagccaccuuguggaauccu

SEQ ID NO: 342 - RNA, 21 nt, Artificial Sequence
  asiRNA
acaagccaccuuguggaaucc

SEQ ID NO: 343 - RNA, 21 nt, Artificial Sequence
  asiRNA
aacaagccaccuuguggaauc

SEQ ID NO: 344 - RNA, 21 nt, Artificial Sequence
  asiRNA
aaacaagccaccuuguggaau

SEQ ID NO: 345 - RNA, 21 nt, Artificial Sequence
  asiRNA
uaaacaagccaccuuguggaa

SEQ ID NO: 346 - RNA, 21 nt, Artificial Sequence
  asiRNA
guaaacaagccaccuugugga

SEQ ID NO: 347 - RNA, 21 nt, Artificial Sequence
  asiRNA
aggaaauuggcuccagaaaca

SEQ ID NO: 348 - RNA, 21 nt, Artificial Sequence
  asiRNA
ggaaauuggcuccagaaacau

SEQ ID NO: 349 - RNA, 21 nt, Artificial Sequence
  asiRNA
gaaauuggcuccagaaacaua

SEQ ID NO: 350 - RNA, 21 nt, Artificial Sequence
  asiRNA
aaauuggcuccagaaacauac

SEQ ID NO: 351 - RNA, 21 nt, Artificial Sequence
  asiRNA
aauuggcuccagaaacauacg

SEQ ID NO: 352 - RNA, 21 nt, Artificial Sequence
  asiRNA
auuggcuccagaaacauacgu

SEQ ID NO: 353 - RNA, 21 nt, Artificial Sequence
  asiRNA
uuggcuccagaaacauacgua

SEQ ID NO: 354 - RNA, 21 nt, Artificial Sequence
  asiRNA
uggcuccagaaacauacguaa

SEQ ID NO: 355 - RNA, 21 nt, Artificial Sequence
  asiRNA
ggcuccagaaacauacguaaa

SEQ ID NO: 356 - RNA, 21 nt, Artificial Sequence
  asiRNA
gcuccagaaacauacguaaac

SEQ ID NO: 357 - RNA, 21 nt, Artificial Sequence
  asiRNA
ugagguagaaccuaugguggu

SEQ ID NO: 358 - RNA, 21 nt, Artificial Sequence
  asiRNA
uugagguagaaccuauggugg

SEQ ID NO: 359 - RNA, 21 nt, Artificial Sequence
  asiRNA
cuugagguagaaccuauggug

SEQ ID NO: 360 - RNA, 21 nt, Artificial Sequence
  asiRNA
ucuugagguagaaccuauggu

SEQ ID NO: 361 - RNA, 21 nt, Artificial Sequence
  asiRNA
aucuugagguagaaccuaugg

SEQ ID NO: 362 - RNA, 21 nt, Artificial Sequence
  asiRNA
caucuugagguagaaccuaug

SEQ ID NO: 363 - RNA, 21 nt, Artificial Sequence
  asiRNA
acaucuugagguagaaccuau

SEQ ID NO: 364 - RNA, 21 nt, Artificial Sequence
  asiRNA
aacaucuugagguagaaccua

SEQ ID NO: 365 - RNA, 21 nt, Artificial Sequence
  asiRNA
ggcuuuccgagauuuggggua

SEQ ID NO: 366 - RNA, 21 nt, Artificial Sequence
  asiRNA
gggcuuuccgagauuuggggu

SEQ ID NO: 367 - RNA, 21 nt, Artificial Sequence
  asiRNA
agggcuuuccgagauuugggg

SEQ ID NO: 368 - RNA, 21 nt, Artificial Sequence
  asiRNA
ugaauggaauaagggcuuucc

SEQ ID NO: 369 - RNA, 21 nt, Artificial Sequence
  asiRNA
augaauggaauaagggcuuuc

SEQ ID NO: 370 - RNA, 21 nt, Artificial Sequence
  asiRNA
gaugaauggaauaagggcuuu

SEQ ID NO: 371 - RNA, 21 nt, Artificial Sequence
  asiRNA
agaugaauggaauaagggcuu

SEQ ID NO: 372 - RNA, 21 nt, Artificial Sequence
  asiRNA
aagaugaauggaauaagggcu

SEQ ID NO: 373 - RNA, 21 nt, Artificial Sequence
  asiRNA
aaagaugaauggaauaagggc

SEQ ID NO: 374 - RNA, 21 nt, Artificial Sequence
  asiRNA
aaaagaugaauggaauaaggg

SEQ ID NO: 375 - RNA, 21 nt, Artificial Sequence
  asiRNA
uaaaagaugaauggaauaagg

SEQ ID NO: 376 - RNA, 21 nt, Artificial Sequence
  asiRNA
uuaaaagaugaauggaauaag

SEQ ID NO: 377 - RNA, 21 nt, Artificial Sequence
  asiRNA
aggaaacaaagugagaaaaau

SEQ ID NO: 378 - RNA, 21 nt, Artificial Sequence
  asiRNA
ggaaacaaagugagaaaaaug

SEQ ID NO: 379 - RNA, 21 nt, Artificial Sequence
  asiRNA
gaaacaaagugagaaaaaugc

SEQ ID NO: 380 - RNA, 21 nt, Artificial Sequence
  asiRNA
aaacaaagugagaaaaaugca

SEQ ID NO: 381 - RNA, 21 nt, Artificial Sequence
  asiRNA
aacaaagugagaaaaaugcaa

SEQ ID NO: 382 - RNA, 21 nt, Artificial Sequence
  asiRNA
acaaagugagaaaaaugcaaa

SEQ ID NO: 383 - RNA, 21 nt, Artificial Sequence
  asiRNA
guggcgcugccugccagcacu

SEQ ID NO: 384 - RNA, 21 nt, Artificial Sequence
  asiRNA
uggcgcugccugccagcacug

SEQ ID NO: 385 - RNA, 21 nt, Artificial Sequence
  asiRNA
aguggcgcugccugccagcac

SEQ ID NO: 386 - RNA, 21 nt, Artificial Sequence
  asiRNA
gcggcgcgggcuggcaggcgg

SEQ ID NO: 387 - RNA, 21 nt, Artificial Sequence
  asiRNA
uguccuguggaaguaauguag

SEQ ID NO: 388 - RNA, 21 nt, Artificial Sequence
  asiRNA
ccuacauuacuuccacaggac

SEQ ID NO: 389 - RNA, 21 nt, Artificial Sequence
  asiRNA
guaccacccaucaggguauuc

SEQ ID NO: 390 - RNA, 21 nt, Artificial Sequence
  asiRNA
uguaccacccaucaggguauu

SEQ ID NO: 391 - RNA, 21 nt, Artificial Sequence
  asiRNA
guguaccacccaucaggguau

SEQ ID NO: 392 - RNA, 21 nt, Artificial Sequence
  asiRNA
uguguaccacccaucagggua

SEQ ID NO: 393 - RNA, 21 nt, Artificial Sequence
  asiRNA
cuguguaccacccaucagggu

SEQ ID NO: 394 - RNA, 21 nt, Artificial Sequence
  asiRNA
ucuguguaccacccaucaggg

SEQ ID NO: 395 - RNA, 21 nt, Artificial Sequence
  asiRNA
gucuguguaccacccaucagg

SEQ ID NO: 396 - RNA, 21 nt, Artificial Sequence
  asiRNA
ugucuguguaccacccaucag

SEQ ID NO: 397 - RNA, 21 nt, Artificial Sequence
  asiRNA
augucuguguaccacccauca

SEQ ID NO: 398 - RNA, 21 nt, Artificial Sequence
  asiRNA
agcuaaaccguaugucugugu

SEQ ID NO: 399 - RNA, 21 nt, Artificial Sequence
  asiRNA
uaagaagacacccaagcuaaa

SEQ ID NO: 400 - RNA, 21 nt, Artificial Sequence
  asiRNA
aagaagacacccaagcuaaac

SEQ ID NO: 401 - RNA, 21 nt, Artificial Sequence
  asiRNA
agaagacacccaagcuaaacc

SEQ ID NO: 402 - RNA, 21 nt, Artificial Sequence
  asiRNA
gaagacacccaagcuaaaccg

SEQ ID NO: 403 - RNA, 21 nt, Artificial Sequence
  asiRNA
ggcuuccugagcuggcgcaau

SEQ ID NO: 404 - RNA, 21 nt, Artificial Sequence
  asiRNA
gcuuccugagcuggcgcaaua

SEQ ID NO: 405 - RNA, 21 nt, Artificial Sequence
  asiRNA
cuuccugagcuggcgcaauau

SEQ ID NO: 406 - RNA, 21 nt, Artificial Sequence
  asiRNA
gaggaaauuggcuccagaaac

SEQ ID NO: 407 - RNA, 21 nt, Artificial Sequence
  asiRNA
aaggaaacaaagugagaaaaa

SEQ ID NO: 408 - RNA, 21 nt, Artificial Sequence
  asiRNA
caaagugagaaaaaugcaaau

SEQ ID NO: 409 - RNA, 21 nt, Artificial Sequence
  asiRNA
gagguagaaccuaugguggug

SEQ ID NO: 410 - RNA, 21 nt, Artificial Sequence
  asiRNA
agguagaaccuauggugguga

SEQ ID NO: 411 - RNA, 21 nt, Artificial Sequence
  asiRNA
gguagaaccuaugguggugaa

SEQ ID NO: 412 - RNA, 21 nt, Artificial Sequence
  asiRNA
guagaaccuaugguggugaaa

SEQ ID NO: 413 - RNA, 21 nt, Artificial Sequence
  asiRNA
uagaaccuaugguggugaaaa

SEQ ID NO: 414 - RNA, 21 nt, Artificial Sequence
  asiRNA
agaaccuaugguggugaaaag

SEQ ID NO: 415 - RNA, 21 nt, Artificial Sequence
  asiRNA
agauuugggguaguccucaaa

SEQ ID NO: 416 - RNA, 21 nt, Artificial Sequence
  asiRNA
gauuugggguaguccucaaac

SEQ ID NO: 417 - RNA, 21 nt, Artificial Sequence
  asiRNA
auuugggguaguccucaaaca

SEQ ID NO: 418 - RNA, 21 nt, Artificial Sequence
  asiRNA
uuugggguaguccucaaacau

SEQ ID NO: 419 - RNA, 21 nt, Artificial Sequence
  asiRNA
uugggguaguccucaaacauc

SEQ ID NO: 420 - RNA, 21 nt, Artificial Sequence
  asiRNA
ugggguaguccucaaacaucu

SEQ ID NO: 421 - RNA, 21 nt, Artificial Sequence
  asiRNA
gcuuuccgagauuugggguag

SEQ ID NO: 422 - RNA, 21 nt, Artificial Sequence
  asiRNA
gaauggaauaagggcuuuccg

SEQ ID NO: 423 - RNA, 21 nt, Artificial Sequence
  asiRNA
aauggaauaagggcuuuccga

SEQ ID NO: 424 - RNA, 21 nt, Artificial Sequence
  asiRNA
uggccagggcauagccgaucc

SEQ ID NO: 425 - DNA, 20 bp, Artificial Sequence
  Primer
gagtcaacggatttggtcgt

SEQ ID NO: 426 - DNA, 20 bp, Artificial Sequence
  Primer
gacaagcttcccgttctcag

SEQ ID NO: 427 - DNA, 20 bp, Artificial Sequence
  Primer
tgaacctgggtggcttatga

SEQ ID NO: 428 - DNA, 19 bp, Artificial Sequence
  Primer
gaaaggaaagttgcttggg

SEQ ID NO: 429 - RNA, 16 nt, Artificial Sequence
  asiRNA
gagaugaagcuucugg

SEQ ID NO: 430 - RNA, 16 nt, Artificial Sequence
  asiRNA
ggagaugaagcuucug

SEQ ID NO: 431 - RNA, 16 nt, Artificial Sequence
  asiRNA
guggagaugaagcuuc

SEQ ID NO: 432 - RNA, 16 nt, Artificial Sequence
  asiRNA
uguggagaugaagcuu

SEQ ID NO: 433 - RNA, 16 nt, Artificial Sequence
  asiRNA
ucuguggagaugaagc

SEQ ID NO: 434 - RNA, 16 nt, Artificial Sequence
  asiRNA
ugaucuguggagauga

SEQ ID NO: 435 - RNA, 16 nt, Artificial Sequence
  asiRNA
cugaucuguggagaug

SEQ ID NO: 436 - RNA, 16 nt, Artificial Sequence
  asiRNA
aagaccugccugaucu

SEQ ID NO: 437 - RNA, 16 nt, Artificial Sequence
  asiRNA
uuuccaccccagaaga

SEQ ID NO: 438 - RNA, 16 nt, Artificial Sequence
  asiRNA
acuuuccaccccagaa

SEQ ID NO: 439 - RNA, 16 nt, Artificial Sequence
  asiRNA
aagggaaacagaagua

SEQ ID NO: 440 - RNA, 16 nt, Artificial Sequence
  asiRNA
gaagggaaacagaagu

SEQ ID NO: 441 - RNA, 16 nt, Artificial Sequence
  asiRNA
cugaagggaaacagaa

SEQ ID NO: 442 - RNA, 16 nt, Artificial Sequence
  asiRNA
caaaagagccgcugaa

SEQ ID NO: 443 - RNA, 16 nt, Artificial Sequence
  asiRNA
ucaaaagagccgcuga

SEQ ID NO: 444 - RNA, 16 nt, Artificial Sequence
  asiRNA
cuucaaaagagccgcu

SEQ ID NO: 445 - RNA, 16 nt, Artificial Sequence
  asiRNA
cuucuucaaaagagcc

SEQ ID NO: 446 - RNA, 16 nt, Artificial Sequence
  asiRNA
ucuucuucaaaagagc

SEQ ID NO: 447 - RNA, 16 nt, Artificial Sequence
  asiRNA
aggucuucuucaaaag

SEQ ID NO: 448 - RNA, 16 nt, Artificial Sequence
  asiRNA
aagcagggaugacucu

SEQ ID NO: 449 - RNA, 16 nt, Artificial Sequence
  asiRNA
ugaagcagggaugacu

SEQ ID NO: 450 - RNA, 16 nt, Artificial Sequence
  asiRNA
uuaugaagcagggaug

SEQ ID NO: 451 - RNA, 16 nt, Artificial Sequence
  asiRNA
uguuaugaagcaggga

SEQ ID NO: 452 - RNA, 16 nt, Artificial Sequence
  asiRNA
auguuaugaagcaggg

SEQ ID NO: 453 - RNA, 16 nt, Artificial Sequence
  asiRNA
gcuaugaaugucagcc

SEQ ID NO: 454 - RNA, 16 nt, Artificial Sequence
  asiRNA
ggcuaugaaugucagc

SEQ ID NO: 455 - RNA, 16 nt, Artificial Sequence
  asiRNA
gaaggcuaugaauguc

SEQ ID NO: 456 - RNA, 16 nt, Artificial Sequence
  asiRNA
uugaaggcuaugaaug

SEQ ID NO: 457 - RNA, 16 nt, Artificial Sequence
  asiRNA
gaagccauugagccag

SEQ ID NO: 458 - RNA, 16 nt, Artificial Sequence
  asiRNA
cuggcuuccgcaacuu

SEQ ID NO: 459 - RNA, 16 nt, Artificial Sequence
  asiRNA
ugccuggcuuccgcaa

SEQ ID NO: 460 - RNA, 16 nt, Artificial Sequence
  asiRNA
agugggccaaggccuu

SEQ ID NO: 461 - RNA, 16 nt, Artificial Sequence
  asiRNA
ccaggaugcucuacuu

SEQ ID NO: 462 - RNA, 16 nt, Artificial Sequence
  asiRNA
uccaggaugcucuacu

SEQ ID NO: 463 - RNA, 16 nt, Artificial Sequence
  asiRNA
aacuccaggaugcucu

SEQ ID NO: 464 - RNA, 16 nt, Artificial Sequence
  asiRNA
uaccgcaugcacaagu

SEQ ID NO: 465 - RNA, 16 nt, Artificial Sequence
  asiRNA
aguaccgcaugcacaa

SEQ ID NO: 466 - RNA, 16 nt, Artificial Sequence
  asiRNA
caaugaguaccgcaug

SEQ ID NO: 467 - RNA, 16 nt, Artificial Sequence
  asiRNA
ucaaugaguaccgcau

SEQ ID NO: 468 - RNA, 16 nt, Artificial Sequence
  asiRNA
uucaaugaguaccgca

SEQ ID NO: 469 - RNA, 16 nt, Artificial Sequence
  asiRNA
uuggauggcuccaaau

SEQ ID NO: 470 - RNA, 16 nt, Artificial Sequence
  asiRNA
aguuuggauggcucca

SEQ ID NO: 471 - RNA, 16 nt, Artificial Sequence
  asiRNA
agaguuuggauggcuc

SEQ ID NO: 472 - RNA, 16 nt, Artificial Sequence
  asiRNA
ucaaggaacucgaucg

SEQ ID NO: 473 - RNA, 16 nt, Artificial Sequence
  asiRNA
caucaaggaacucgau

SEQ ID NO: 474 - RNA, 16 nt, Artificial Sequence
  asiRNA
cuacaucaaggaacuc

SEQ ID NO: 475 - RNA, 16 nt, Artificial Sequence
  asiRNA
gaacuacaucaaggaa

SEQ ID NO: 476 - RNA, 16 nt, Artificial Sequence
  asiRNA
cuucgaaugaacuaca

SEQ ID NO: 477 - RNA, 16 nt, Artificial Sequence
  asiRNA
ugaacuucgaaugaac

SEQ ID NO: 478 - RNA, 16 nt, Artificial Sequence
  asiRNA
ugaugaacuucgaaug

SEQ ID NO: 479 - RNA, 16 nt, Artificial Sequence
  asiRNA
gggcugaaaaaucaaa

SEQ ID NO: 480 - RNA, 16 nt, Artificial Sequence
  asiRNA
gaugggcugaaaaauc

SEQ ID NO: 481 - RNA, 16 nt, Artificial Sequence
  asiRNA
uauuccaguggauggg

SEQ ID NO: 482 - RNA, 16 nt, Artificial Sequence
  asiRNA
cauuauuccaguggau

SEQ ID NO: 483 - RNA, 16 nt, Artificial Sequence
  asiRNA
agcauuauuccagugg

SEQ ID NO: 484 - RNA, 16 nt, Artificial Sequence
  asiRNA
uucagcauuauuccag

SEQ ID NO: 485 - RNA, 16 nt, Artificial Sequence
  asiRNA
cucuucagcauuauuc

SEQ ID NO: 486 - RNA, 16 nt, Artificial Sequence
  asiRNA
cugcucucuucagcau

SEQ ID NO: 487 - RNA, 16 nt, Artificial Sequence
  asiRNA
aagcacugcucucuuc

SEQ ID NO: 488 - RNA, 16 nt, Artificial Sequence
  asiRNA
gaaagcacugcucucu

SEQ ID NO: 489 - RNA, 16 nt, Artificial Sequence
  asiRNA
caugaaagcacugcuc

SEQ ID NO: 490 - RNA, 16 nt, Artificial Sequence
  asiRNA
gugcaugaaagcacug

SEQ ID NO: 491 - RNA, 16 nt, Artificial Sequence
  asiRNA
uuccugugcaugaaag

SEQ ID NO: 492 - RNA, 16 nt, Artificial Sequence
  asiRNA
gaauuccugugcauga

SEQ ID NO: 493 - RNA, 16 nt, Artificial Sequence
  asiRNA
aggaauuccugugcau

SEQ ID NO: 494 - RNA, 16 nt, Artificial Sequence
  asiRNA
ucaccaagcuccugga

SEQ ID NO: 495 - RNA, 16 nt, Artificial Sequence
  asiRNA
accagcucaccaagcu

SEQ ID NO: 496 - RNA, 16 nt, Artificial Sequence
  asiRNA
cuaccagcucaccaag

SEQ ID NO: 497 - RNA, 16 nt, Artificial Sequence
  asiRNA
accugcuaaucaaguc

SEQ ID NO: 498 - RNA, 16 nt, Artificial Sequence
  asiRNA
gaccugcuaaucaagu

SEQ ID NO: 499 - RNA, 16 nt, Artificial Sequence
  asiRNA
uuugaccugcuaauca

SEQ ID NO: 500 - RNA, 16 nt, Artificial Sequence
  asiRNA
cuuuugaccugcuaau

SEQ ID NO: 501 - RNA, 16 nt, Artificial Sequence
  asiRNA
ucacuuuugaccugcu

SEQ ID NO: 502 - RNA, 16 nt, Artificial Sequence
  asiRNA
uucacuuuugaccugc

SEQ ID NO: 503 - RNA, 16 nt, Artificial Sequence
  asiRNA
caguucacuuuugacc

SEQ ID NO: 504 - RNA, 16 nt, Artificial Sequence
  asiRNA
caucaguucacuuuug

SEQ ID NO: 505 - RNA, 16 nt, Artificial Sequence
  asiRNA
cugcaucaguucacuu

SEQ ID NO: 506 - RNA, 16 nt, Artificial Sequence
  asiRNA
gcugcaucaguucacu

SEQ ID NO: 507 - RNA, 16 nt, Artificial Sequence
  asiRNA
ccaucuauuuccacac

SEQ ID NO: 508 - RNA, 16 nt, Artificial Sequence
  asiRNA
cccaucuauuuccaca

SEQ ID NO: 509 - RNA, 16 nt, Artificial Sequence
  asiRNA
agcccaucuauuucca

SEQ ID NO: 510 - RNA, 16 nt, Artificial Sequence
  asiRNA
ucaagcccaucuauuu

SEQ ID NO: 511 - RNA, 16 nt, Artificial Sequence
  asiRNA
ggaaagucaagcccau

SEQ ID NO: 512 - RNA, 16 nt, Artificial Sequence
  asiRNA
cugggaaagucaagcc

SEQ ID NO: 513 - RNA, 16 nt, Artificial Sequence
  asiRNA
uuucugggaaagucaa

SEQ ID NO: 514 - RNA, 16 nt, Artificial Sequence
  asiRNA
uccuuucugggaaagu

SEQ ID NO: 515 - RNA, 16 nt, Artificial Sequence
  asiRNA
ccaagauccuuucugg

SEQ ID NO: 516 - RNA, 16 nt, Artificial Sequence
  asiRNA
ugcccaagauccuuuc

SEQ ID NO: 517 - RNA, 16 nt, Artificial Sequence
  asiRNA
aagugcccaagauccu

SEQ ID NO: 518 - RNA, 16 nt, Artificial Sequence
  asiRNA
ugcaagugcccaagau

SEQ ID NO: 519 - RNA, 16 nt, Artificial Sequence
  asiRNA
ucucugugcaagugcc

SEQ ID NO: 520 - RNA, 16 nt, Artificial Sequence
  asiRNA
ucaucucugugcaagu

SEQ ID NO: 521 - RNA, 16 nt, Artificial Sequence
  asiRNA
agaucaucucugugca

SEQ ID NO: 522 - RNA, 16 nt, Artificial Sequence
  asiRNA
cagagaucaucucugu

SEQ ID NO: 523 - RNA, 16 nt, Artificial Sequence
  asiRNA
cacuggcacuaaaaaa

SEQ ID NO: 524 - RNA, 16 nt, Artificial Sequence
  asiRNA
ucacuggcacuaaaaa

SEQ ID NO: 525 - RNA, 16 nt, Artificial Sequence
  asiRNA
guucacuggcacuaaa

SEQ ID NO: 526 - RNA, 16 nt, Artificial Sequence
  asiRNA
uauguucacuggcacu

SEQ ID NO: 527 - RNA, 16 nt, Artificial Sequence
  asiRNA
uguauguucacuggca

SEQ ID NO: 528 - RNA, 16 nt, Artificial Sequence
  asiRNA
uauguauguucacugg

SEQ ID NO: 529 - RNA, 16 nt, Artificial Sequence
  asiRNA
ggguaguugcugaggu

SEQ ID NO: 530 - RNA, 16 nt, Artificial Sequence
  asiRNA
uggguaguugcugagg

SEQ ID NO: 531 - RNA, 16 nt, Artificial Sequence
  asiRNA
cuuuggguaguugcug

SEQ ID NO: 532 - RNA, 16 nt, Artificial Sequence
  asiRNA
ccuuuggguaguugcu

SEQ ID NO: 533 - RNA, 16 nt, Artificial Sequence
  asiRNA
ccaccauccacaugau

SEQ ID NO: 534 - RNA, 16 nt, Artificial Sequence
  asiRNA
cauuagugccucuuug

SEQ ID NO: 535 - RNA, 16 nt, Artificial Sequence
  asiRNA
gcauuagugccucuuu

SEQ ID NO: 536 - RNA, 16 nt, Artificial Sequence
  asiRNA
agcauuagugccucuu

SEQ ID NO: 537 - RNA, 16 nt, Artificial Sequence
  asiRNA
aagcauuagugccucu

SEQ ID NO: 538 - RNA, 16 nt, Artificial Sequence
  asiRNA
gcccauguuagcuuau

SEQ ID NO: 539 - RNA, 16 nt, Artificial Sequence
  asiRNA
gaaacuuguuuguugg

SEQ ID NO: 540 - RNA, 16 nt, Artificial Sequence
  asiRNA
gcagaaacuuguuugu

SEQ ID NO: 541 - RNA, 16 nt, Artificial Sequence
  asiRNA
auggcagaaacuuguu

SEQ ID NO: 542 - RNA, 16 nt, Artificial Sequence
  asiRNA
aauggcagaaacuugu

SEQ ID NO: 543 - RNA, 16 nt, Artificial Sequence
  asiRNA
ggaaucuuuuguugcu

SEQ ID NO: 544 - RNA, 16 nt, Artificial Sequence
  asiRNA
uggaaucuuuuguugc

SEQ ID NO: 545 - RNA, 16 nt, Artificial Sequence
  asiRNA
uaguguucuguucucu

SEQ ID NO: 546 - RNA, 16 nt, Artificial Sequence
  asiRNA
cuaguguucuguucuc

SEQ ID NO: 547 - RNA, 21 nt, Artificial Sequence
  asiRNA
ccagaagcuucaucuccacag

SEQ ID NO: 548 - RNA, 21 nt, Artificial Sequence
  asiRNA
cagaagcuucaucuccacaga

SEQ ID NO: 549 - RNA, 21 nt, Artificial Sequence
  asiRNA
gaagcuucaucuccacagauc

SEQ ID NO: 550 - RNA, 21 nt, Artificial Sequence
  asiRNA
aagcuucaucuccacagauca

SEQ ID NO: 551 - RNA, 21 nt, Artificial Sequence
  asiRNA
gcuucaucuccacagaucagg

SEQ ID NO: 552 - RNA, 21 nt, Artificial Sequence
  asiRNA
ucaucuccacagaucaggcag

SEQ ID NO: 553 - RNA, 21 nt, Artificial Sequence
  asiRNA
caucuccacagaucaggcagg

SEQ ID NO: 554 - RNA, 21 nt, Artificial Sequence
  asiRNA
agaucaggcaggucuucuggg

SEQ ID NO: 555 - RNA, 21 nt, Artificial Sequence
  asiRNA
ucuucugggguggaaaguaau

SEQ ID NO: 556 - RNA, 21 nt, Artificial Sequence
  asiRNA
uucugggguggaaaguaauag

SEQ ID NO: 557 - RNA, 21 nt, Artificial Sequence
  asiRNA
uacuucuguuucccuucagcg

SEQ ID NO: 558 - RNA, 21 nt, Artificial Sequence
  asiRNA
acuucuguuucccuucagcgg

SEQ ID NO: 559 - RNA, 21 nt, Artificial Sequence
  asiRNA
uucuguuucccuucagcggcu

SEQ ID NO: 560 - RNA, 21 nt, Artificial Sequence
  asiRNA
uucagcggcucuuuugaagaa

SEQ ID NO: 561 - RNA, 21 nt, Artificial Sequence
  asiRNA
ucagcggcucuuuugaagaag

SEQ ID NO: 562 - RNA, 21 nt, Artificial Sequence
  asiRNA
agcggcucuuuugaagaagac

SEQ ID NO: 563 - RNA, 21 nt, Artificial Sequence
  asiRNA
ggcucuuuugaagaagaccuu

SEQ ID NO: 564 - RNA, 21 nt, Artificial Sequence
  asiRNA
gcucuuuugaagaagaccuug

SEQ ID NO: 565 - RNA, 21 nt, Artificial Sequence
  asiRNA
cuuuugaagaagaccuugcag

SEQ ID NO: 566 - RNA, 21 nt, Artificial Sequence
  asiRNA
agagucaucccugcuucauaa

SEQ ID NO: 567 - RNA, 21 nt, Artificial Sequence
  asiRNA
agucaucccugcuucauaaca

SEQ ID NO: 568 - RNA, 21 nt, Artificial Sequence
  asiRNA
caucccugcuucauaacauuu

SEQ ID NO: 569 - RNA, 21 nt, Artificial Sequence
  asiRNA
ucccugcuucauaacauuucc

SEQ ID NO: 570 - RNA, 21 nt, Artificial Sequence
  asiRNA
cccugcuucauaacauuuccg

SEQ ID NO: 571 - RNA, 21 nt, Artificial Sequence
  asiRNA
ggcugacauucauagccuuca

SEQ ID NO: 572 - RNA, 21 nt, Artificial Sequence
  asiRNA
gcugacauucauagccuucaa

SEQ ID NO: 573 - RNA, 21 nt, Artificial Sequence
  asiRNA
gacauucauagccuucaaugu

SEQ ID NO: 574 - RNA, 21 nt, Artificial Sequence
  asiRNA
cauucauagccuucaaugugu

SEQ ID NO: 575 - RNA, 21 nt, Artificial Sequence
  asiRNA
cuggcucaauggcuuccagga

SEQ ID NO: 576 - RNA, 21 nt, Artificial Sequence
  asiRNA
aaguugcggaagccaggcaag

SEQ ID NO: 577 - RNA, 21 nt, Artificial Sequence
  asiRNA
uugcggaagccaggcaaggcc

SEQ ID NO: 578 - RNA, 21 nt, Artificial Sequence
  asiRNA
aaggccuuggcccacuugacc

SEQ ID NO: 579 - RNA, 21 nt, Artificial Sequence
  asiRNA
aaguagagcauccuggaguug

SEQ ID NO: 580 - RNA, 21 nt, Artificial Sequence
  asiRNA
aguagagcauccuggaguuga

SEQ ID NO: 581 - RNA, 21 nt, Artificial Sequence
  asiRNA
agagcauccuggaguugacau

SEQ ID NO: 582 - RNA, 21 nt, Artificial Sequence
  asiRNA
acuugugcaugcgguacucau

SEQ ID NO: 583 - RNA, 21 nt, Artificial Sequence
  asiRNA
uugugcaugcgguacucauug

SEQ ID NO: 584 - RNA, 21 nt, Artificial Sequence
  asiRNA
caugcgguacucauugaaaac

SEQ ID NO: 585 - RNA, 21 nt, Artificial Sequence
  asiRNA
augcgguacucauugaaaacc

SEQ ID NO: 586 - RNA, 21 nt, Artificial Sequence
  asiRNA
ugcgguacucauugaaaacca

SEQ ID NO: 587 - RNA, 21 nt, Artificial Sequence
  asiRNA
auuuggagccauccaaacucu

SEQ ID NO: 588 - RNA, 21 nt, Artificial Sequence
  asiRNA
uggagccauccaaacucuuga

SEQ ID NO: 589 - RNA, 21 nt, Artificial Sequence
  asiRNA
gagccauccaaacucuugaga

SEQ ID NO: 590 - RNA, 21 nt, Artificial Sequence
  asiRNA
cgaucgaguuccuugauguag

SEQ ID NO: 591 - RNA, 21 nt, Artificial Sequence
  asiRNA
aucgaguuccuugauguaguu

SEQ ID NO: 592 - RNA, 21 nt, Artificial Sequence
  asiRNA
gaguuccuugauguaguucau

SEQ ID NO: 593 - RNA, 21 nt, Artificial Sequence
  asiRNA
uuccuugauguaguucauucg

SEQ ID NO: 594 - RNA, 21 nt, Artificial Sequence
  asiRNA
uguaguucauucgaaguucau

SEQ ID NO: 595 - RNA, 21 nt, Artificial Sequence
  asiRNA
guucauucgaaguucaucaaa

SEQ ID NO: 596 - RNA, 21 nt, Artificial Sequence
  asiRNA
cauucgaaguucaucaaagaa

SEQ ID NO: 597 - RNA, 21 nt, Artificial Sequence
  asiRNA
uuugauuuuucagcccaucca

SEQ ID NO: 598 - RNA, 21 nt, Artificial Sequence
  asiRNA
gauuuuucagcccauccacug

SEQ ID NO: 599 - RNA, 21 nt, Artificial Sequence
  asiRNA
cccauccacuggaauaaugcu

SEQ ID NO: 600 - RNA, 21 nt, Artificial Sequence
  asiRNA
auccacuggaauaaugcugaa

SEQ ID NO: 601 - RNA, 21 nt, Artificial Sequence
  asiRNA
ccacuggaauaaugcugaaga

SEQ ID NO: 602 - RNA, 21 nt, Artificial Sequence
  asiRNA
cuggaauaaugcugaagagag

SEQ ID NO: 603 - RNA, 21 nt, Artificial Sequence
  asiRNA
gaauaaugcugaagagagcag

SEQ ID NO: 604 - RNA, 21 nt, Artificial Sequence
  asiRNA
augcugaagagagcagugcuu

SEQ ID NO: 605 - RNA, 21 nt, Artificial Sequence
  asiRNA
gaagagagcagugcuuucaug

SEQ ID NO: 606 - RNA, 21 nt, Artificial Sequence
  asiRNA
agagagcagugcuuucaugca

SEQ ID NO: 607 - RNA, 21 nt, Artificial Sequence
  asiRNA
gagcagugcuuucaugcacag

SEQ ID NO: 608 - RNA, 21 nt, Artificial Sequence
  asiRNA
cagugcuuucaugcacaggaa

SEQ ID NO: 609 - RNA, 21 nt, Artificial Sequence
  asiRNA
cuuucaugcacaggaauuccu

SEQ ID NO: 610 - RNA, 21 nt, Artificial Sequence
  asiRNA
ucaugcacaggaauuccuggg

SEQ ID NO: 611 - RNA, 21 nt, Artificial Sequence
  asiRNA
augcacaggaauuccuggggg

SEQ ID NO: 612 - RNA, 21 nt, Artificial Sequence
  asiRNA
uccaggagcuuggugagcugg

SEQ ID NO: 613 - RNA, 21 nt, Artificial Sequence
  asiRNA
agcuuggugagcugguagaag

SEQ ID NO: 614 - RNA, 21 nt, Artificial Sequence
  asiRNA
cuuggugagcugguagaagcg

SEQ ID NO: 615 - RNA, 21 nt, Artificial Sequence
  asiRNA
gacuugauuagcaggucaaaa

SEQ ID NO: 616 - RNA, 21 nt, Artificial Sequence
  asiRNA
acuugauuagcaggucaaaag

SEQ ID NO: 617 - RNA, 21 nt, Artificial Sequence
  asiRNA
ugauuagcaggucaaaaguga

SEQ ID NO: 618 - RNA, 21 nt, Artificial Sequence
  asiRNA
auuagcaggucaaaagugaac

SEQ ID NO: 619 - RNA, 21 nt, Artificial Sequence
  asiRNA
agcaggucaaaagugaacuga

SEQ ID NO: 620 - RNA, 21 nt, Artificial Sequence
  asiRNA
gcaggucaaaagugaacugau

SEQ ID NO: 621 - RNA, 21 nt, Artificial Sequence
  asiRNA
ggucaaaagugaacugaugca

SEQ ID NO: 622 - RNA, 21 nt, Artificial Sequence
  asiRNA
caaaagugaacugaugcagcu

SEQ ID NO: 623 - RNA, 21 nt, Artificial Sequence
  asiRNA
aagugaacugaugcagcucuc

SEQ ID NO: 624 - RNA, 21 nt, Artificial Sequence
  asiRNA
agugaacugaugcagcucucu

SEQ ID NO: 625 - RNA, 21 nt, Artificial Sequence
  asiRNA
guguggaaauagaugggcuug

SEQ ID NO: 626 - RNA, 21 nt, Artificial Sequence
  asiRNA
uguggaaauagaugggcuuga

SEQ ID NO: 627 - RNA, 21 nt, Artificial Sequence
  asiRNA
uggaaauagaugggcuugacu

SEQ ID NO: 628 - RNA, 21 nt, Artificial Sequence
  asiRNA
aaauagaugggcuugacuuuc

SEQ ID NO: 629 - RNA, 21 nt, Artificial Sequence
  asiRNA
augggcuugacuuucccagaa

SEQ ID NO: 630 - RNA, 21 nt, Artificial Sequence
  asiRNA
ggcuugacuuucccagaaagg

SEQ ID NO: 631 - RNA, 21 nt, Artificial Sequence
  asiRNA
uugacuuucccagaaaggauc

SEQ ID NO: 632 - RNA, 21 nt, Artificial Sequence
  asiRNA
acuuucccagaaaggaucuug

SEQ ID NO: 633 - RNA, 21 nt, Artificial Sequence
  asiRNA
ccagaaaggaucuugggcacu

SEQ ID NO: 634 - RNA, 21 nt, Artificial Sequence
  asiRNA
gaaaggaucuugggcacuugc

SEQ ID NO: 635 - RNA, 21 nt, Artificial Sequence
  asiRNA
aggaucuugggcacuugcaca

SEQ ID NO: 636 - RNA, 21 nt, Artificial Sequence
  asiRNA
aucuugggcacuugcacagag

SEQ ID NO: 637 - RNA, 21 nt, Artificial Sequence
  asiRNA
ggcacuugcacagagaugauc

SEQ ID NO: 638 - RNA, 21 nt, Artificial Sequence
  asiRNA
acuugcacagagaugaucucu

SEQ ID NO: 639 - RNA, 21 nt, Artificial Sequence
  asiRNA
ugcacagagaugaucucugcc

SEQ ID NO: 640 - RNA, 21 nt, Artificial Sequence
  asiRNA
acagagaugaucucugccauc

SEQ ID NO: 641 - RNA, 21 nt, Artificial Sequence
  asiRNA
uuuuuuagugccagugaacau

SEQ ID NO: 642 - RNA, 21 nt, Artificial Sequence
  asiRNA
uuuuuagugccagugaacaua

SEQ ID NO: 643 - RNA, 21 nt, Artificial Sequence
  asiRNA
uuuagugccagugaacauaca

SEQ ID NO: 644 - RNA, 21 nt, Artificial Sequence
  asiRNA
agugccagugaacauacauaa

SEQ ID NO: 645 - RNA, 21 nt, Artificial Sequence
  asiRNA
ugccagugaacauacauaaaa

SEQ ID NO: 646 - RNA, 21 nt, Artificial Sequence
  asiRNA
ccagugaacauacauaaaaau

SEQ ID NO: 647 - RNA, 21 nt, Artificial Sequence
  asiRNA
accucagcaacuacccaaagg

SEQ ID NO: 648 - RNA, 21 nt, Artificial Sequence
  asiRNA
ccucagcaacuacccaaagga

SEQ ID NO: 649 - RNA, 21 nt, Artificial Sequence
  asiRNA
cagcaacuacccaaaggacag

SEQ ID NO: 650 - RNA, 21 nt, Artificial Sequence
  asiRNA
agcaacuacccaaaggacaga

SEQ ID NO: 651 - RNA, 21 nt, Artificial Sequence
  asiRNA
aucauguggaugguggacaua

SEQ ID NO: 652 - RNA, 21 nt, Artificial Sequence
  asiRNA
caaagaggcacuaaugcuugc

SEQ ID NO: 653 - RNA, 21 nt, Artificial Sequence
  asiRNA
aaagaggcacuaaugcuugcu

SEQ ID NO: 654 - RNA, 21 nt, Artificial Sequence
  asiRNA
aagaggcacuaaugcuugcuc

SEQ ID NO: 655 - RNA, 21 nt, Artificial Sequence
  asiRNA
agaggcacuaaugcuugcucc

SEQ ID NO: 656 - RNA, 21 nt, Artificial Sequence
  asiRNA
auaagcuaacaugggcacuag

SEQ ID NO: 657 - RNA, 21 nt, Artificial Sequence
  asiRNA
ccaacaaacaaguuucugcca

SEQ ID NO: 658 - RNA, 21 nt, Artificial Sequence
  asiRNA
acaaacaaguuucugccauuu

SEQ ID NO: 659 - RNA, 21 nt, Artificial Sequence
  asiRNA
aacaaguuucugccauuuuua

SEQ ID NO: 660 - RNA, 21 nt, Artificial Sequence
  asiRNA
acaaguuucugccauuuuuaa

SEQ ID NO: 661 - RNA, 21 nt, Artificial Sequence
  asiRNA
agcaacaaaagauuccaagau

SEQ ID NO: 662 - RNA, 21 nt, Artificial Sequence
  asiRNA
gcaacaaaagauuccaagauu

SEQ ID NO: 663 - RNA, 21 nt, Artificial Sequence
  asiRNA
agagaacagaacacuagcgcu

SEQ ID NO: 664 - RNA, 21 nt, Artificial Sequence
  asiRNA
gagaacagaacacuagcgcuu

SEQ ID NO: 665 - DNA, 20 bp, Artificial Sequence
  Primer
gagtcaacggatttggtcgt

SEQ ID NO: 666 - DNA, 20 bp, Artificial Sequence
  Primer
gacaagcttcccgttctcag

SEQ ID NO: 667 - DNA, 20 bp, Artificial Sequence
  Primer
ggggctagactgctcaactg

SEQ ID NO: 668 - DNA, 20 bp, Artificial Sequence
  Primer
gccaagttttggctgaagag

SEQ ID NO: 669 - DNA, 2350 bp, Artificial Sequence
  NCBI Reference Sequence NM_001047.3
ttactgcggccccggcgtgggtggggcgcttgcaggtccctccccgcgcaagtgctcgccccgcccccggggccgcacccacagccccggctaccccggagaagcctgacttgagaaccctttctgcagagtcccggcagtgcgggactccggtagccgcccctccggtagccgcccctcctgcccccgcgccgccgccctatatgttgcccgccgcggcctctggggcatggagcacgctgcccagccctggcgatggcaacggcgacgggggtggcggaggagcgcctgctggccgcgctcgcctacctgcagtgcgccgtgggctgcgcggtcttcgcgcgcaatcgtcagacgaactcagtgtacggccgccacgcgctgcccagccacaggctccgagtgccggcgcgggccgcctgggtggtgcaggagctgccctcgctggccctgccgctctaccagtacgccagcgagtccgccccgcgtctccgcagcgcgcccaactgcatcctcctggccatgttcctcgtccactacgggcatcggtgcttaatttacccatttctgatgcgaggaggaaagcctatgccactgttggcgtgtacaatggcgattatgttctgtacctgtaacggctatttgcaaagcagatacttgagccattgtgcagtgtatgctgatgactgggtaacagatccccgttttctaataggttttggcttgtggttaacgggcatgttgataaacatccattcagatcatatcctaaggaatctcagaaaaccaggagatactggatacaaaataccaaggggaggcttatttgaatacgtaactgcagccaactattttggagaaatcatggagtggtgtggctatgccctggccagctggtctgtccaaggcgcggcttttgctttcttcacgttttgttttttatctggtagagcaaaagagcatcatgagtggtacctccggaaatttgaagagtatccaaagttcagaaaaattataattccatttttgttttaagtgcgtttttcatgaaattatcttcaacttgaagctttccaatggcgcttctctatggactttgtaaataagttatatctttgtaattttcctgctactttatcattttcaagatgtcctctaggaattttttttctagtaattttgcaatctacctaataagtacctaaatacgctgaaatggaggttgaatatcctactgtgtaacaggtcagaatttcaagctctgggtaataactgctgatattttttctaatttcaaatttacctcttttggctatgtcttgccaagtgtgtatgagactagactttacaactgtctttgatggcattttcagaacaataaatgtcacaatcccttctatagccccctacagtgatctcttcaaggtcaactgcagtgttgcttccctccccctatagggctggaatctgtctaggagccctctctcggaggccacagaggctgggggtagccattgtgcagtcatggcccgggggaaacttgccaaccttcgtgtcaggtgctgtgtgtaagtggagaacttggggatagaggaggaagctcctcgtggcccttccaaggtgaggcaaaggcatctggacttgttccagcccagcccaccgggtgacatcaccgggcagggaggggtgctggtggtggttcatacggagtaagctgctctgcctgtgtgagtggctcctgggccctaaacaggcacctttaggccatgggtcactcaccgtgagccatcaatgtgctctggtctgacatggtttctctctgtcttctagtctagacctagtttttttgttctgttccccacgtatggatatagtagagattgttgtctgtgaaatttctcttttgtagattttgagttttcccttgtagtgtaaagaatgatcactttctgtaacaataacaagaccactttttaagatttatcctgtttgttctttgttgattgaaacataataattgttaaaattctctacagccttctttttcttccatagctaatcttccttctaatagtttttgctttctgttttgctgttgttgctttgcaaagctttcccctcatagcctgtacctgttatcaatataaaataatcttcctgttgaatgcttcatgacttgaattctactttgataaaaacattgccatactgctttttatcttgatgaattcatctggcattgctttgccttatcatctcatctggagtttttaaatgccatttgtttcagttgtctttaacaacataataaatagactttgccatttaaaaaaaaaaaaaaaaaaaaaaa

SEQ ID NO: 670 - DNA, 2183 bp, Artificial Sequence
  NCBI Reference Sequence NM_001324322.1
ttactgcggccccggcgtgggtggggcgcttgcaggtccctccccgcgcaagtgctcgccccgcccccggggccgcacccacagccccggctaccccggagaagcctgacttgagaaccctttctgcagagtcccggcagtgcgggactccggtagccgcccctccggtagccgcccctcctgcccccgcgccgccgccctatatgttgcccgccgcggcctctggggcatggagcacgctgcccagccctggcgatggcaacggcgacgggggtggcggaggagcgcctgctggccgcgctcgcctacctgcagtgcgccgtgggctgcgcggtcttcgcgcgcaatcgtcagacgaactcagtgtacggccgccacgcgctgcccagccacaggctccgagtgccggcgcgggccgcctgggtggtgcaggagctgccctcgctggccctgccgctctaccagtacgccagcgagtccgccccgcgtctccgcagcgcgcccaactgcatcctcctggccatgttcctcgtccactacgggcatcggttttggcttgtggttaacgggcatgttgataaacatccattcagatcatatcctaaggaatctcagaaaaccaggagatactggatacaaaataccaaggggaggcttatttgaatacgtaactgcagccaactattttggagaaatcatggagtggtgtggctatgccctggccagctggtctgtccaaggcgcggcttttgctttcttcacgttttgttttttatctggtagagcaaaagagcatcatgagtggtacctccggaaatttgaagagtatccaaagttcagaaaaattataattccatttttgttttaagtgcgtttttcatgaaattatcttcaacttgaagctttccaatggcgcttctctatggactttgtaaataagttatatctttgtaattttcctgctactttatcattttcaagatgtcctctaggaattttttttctagtaattttgcaatctacctaataagtacctaaatacgctgaaatggaggttgaatatcctactgtgtaacaggtcagaatttcaagctctgggtaataactgctgatattttttctaatttcaaatttacctcttttggctatgtcttgccaagtgtgtatgagactagactttacaactgtctttgatggcattttcagaacaataaatgtcacaatcccttctatagccccctacagtgatctcttcaaggtcaactgcagtgttgcttccctccccctatagggctggaatctgtctaggagccctctctcggaggccacagaggctgggggtagccattgtgcagtcatggcccgggggaaacttgccaaccttcgtgtcaggtgctgtgtgtaagtggagaacttggggatagaggaggaagctcctcgtggcccttccaaggtgaggcaaaggcatctggacttgttccagcccagcccaccgggtgacatcaccgggcagggaggggtgctggtggtggttcatacggagtaagctgctctgcctgtgtgagtggctcctgggccctaaacaggcacctttaggccatgggtcactcaccgtgagccatcaatgtgctctggtctgacatggtttctctctgtcttctagtctagacctagtttttttgttctgttccccacgtatggatatagtagagattgttgtctgtgaaatttctcttttgtagattttgagttttcccttgtagtgtaaagaatgatcactttctgtaacaataacaagaccactttttaagatttatcctgtttgttctttgttgattgaaacataataattgttaaaattctctacagccttctttttcttccatagctaatcttccttctaatagtttttgctttctgttttgctgttgttgctttgcaaagctttcccctcatagcctgtacctgttatcaatataaaataatcttcctgttgaatgcttcatgacttgaattctactttgataaaaacattgccatactgctttttatcttgatgaattcatctggcattgctttgccttatcatctcatctggagtttttaaatgccatttgtttcagttgtctttaacaacataataaatagactttgccatttaaaaaaaaaaaaaaaaaaaaaaa

SEQ ID NO: 671 - DNA, 2852 bp, Artificial Sequence
  NCBI Reference Sequence NM_001324323.1
ttactgcggccccggcgtgggtggggcgcttgcaggtccctccccgcgcaagtgctcgccccgcccccggggccgcacccacagccccggctaccccggagaagcctgacttgagaaccctttctgcagagtcccggcagtgcgggactccggtagccgcccctccggtagccgcccctcctgcccccgcgccgccgccctatatgttgcccgccgcggcctctggggcatggagcacgctgcccagccctggcgatggcaacggcgacgggggtggcggaggagcgcctgctggccgcgctcgcctacctgcagtgcgccgtgggctgcgcggtcttcgcgcgcaatcgtcagacgaactcagtgtacggccgccacgcgctgcccagccacaggctccgagtgccggcgcgggccgcctgggtggtgcaggagctgccctcgctggccctgccgctctaccagtacgccagcgagtccgccccgcgtctccgcagcgcgcccaactgcatcctcctggccatgttcctcgtccactacgggcatcggaaatgttggtatgcaagcacttgcagtgtgcctacatcccaaatgccagcccatggtacccattgtctgcccggatctgaatcatgattccaagacgcagagagaaattgctgggattcgttgttcttattcattgcttggcaacactgcagcttccaggagaatacccacctcactgatgacacaacatctgaatgcacacttactggccaacacgtgctttgctgtaaatcagtatgaagtcttcctaggggtcctggcctgaatgagatgagaaccttggaggctgcttttgactcatgtgaatgtcttccccaggagttaagtgggagtgctggggagagagtggcttgaggatgcacagccagcatgacactactattatgtgattactgtcgacgttcataaccataactaatgactaattatgactttaccctggcgcacatggtcagaatggaaacaaataacaagctttacagtttttcctgctctattaaggtgcttaatttacccatttctgatgcgaggaggaaagcctatgccactgttggcgtgtacaatggcgattatgttctgtacctgtaacggctatttgcaaagcagatacttgagccattgtgcagtgtatgctgatgactgggtaacagatccccgttttctaataggttttggcttgtggttaacgggcatgttgataaacatccattcagatcatatcctaaggaatctcagaaaaccaggagatactggatacaaaataccaaggggaggcttatttgaatacgtaactgcagccaactattttggagaaatcatggagtggtgtggctatgccctggccagctggtctgtccaaggcgcggcttttgctttcttcacgttttgttttttatctggtagagcaaaagagcatcatgagtggtacctccggaaatttgaagagtatccaaagttcagaaaaattataattccatttttgttttaagtgcgtttttcatgaaattatcttcaacttgaagctttccaatggcgcttctctatggactttgtaaataagttatatctttgtaattttcctgctactttatcattttcaagatgtcctctaggaattttttttctagtaattttgcaatctacctaataagtacctaaatacgctgaaatggaggttgaatatcctactgtgtaacaggtcagaatttcaagctctgggtaataactgctgatattttttctaatttcaaatttacctcttttggctatgtcttgccaagtgtgtatgagactagactttacaactgtctttgatggcattttcagaacaataaatgtcacaatcccttctatagccccctacagtgatctcttcaaggtcaactgcagtgttgcttccctccccctatagggctggaatctgtctaggagccctctctcggaggccacagaggctgggggtagccattgtgcagtcatggcccgggggaaacttgccaaccttcgtgtcaggtgctgtgtgtaagtggagaacttggggatagaggaggaagctcctcgtggcccttccaaggtgaggcaaaggcatctggacttgttccagcccagcccaccgggtgacatcaccgggcagggaggggtgctggtggtggttcatacggagtaagctgctctgcctgtgtgagtggctcctgggccctaaacaggcacctttaggccatgggtcactcaccgtgagccatcaatgtgctctggtctgacatggtttctctctgtcttctagtctagacctagtttttttgttctgttccccacgtatggatatagtagagattgttgtctgtgaaatttctcttttgtagattttgagttttcccttgtagtgtaaagaatgatcactttctgtaacaataacaagaccactttttaagatttatcctgtttgttctttgttgattgaaacataataattgttaaaattctctacagccttctttttcttccatagctaatcttccttctaatagtttttgctttctgttttgctgttgttgctttgcaaagctttcccctcatagcctgtacctgttatcaatataaaataatcttcctgttgaatgcttcatgacttgaattctactttgataaaaacattgccatactgctttttatcttgatgaattcatctggcattgctttgccttatcatctcatctggagtttttaaatgccatttgtttcagttgtctttaacaacataataaatagactttgccatttaaaaaaaaaaaaaaaaaaaaaaa

SEQ ID NO: 672 - DNA, 2446 bp, Artificial Sequence
  NCBI Reference Sequence NM_000348.3
tccataaaggggttgcgggggccgcgctctcttctgggagggcagcggccaccggcgaggaacacggcgcgatgcaggttcagtgccagcagagcccagtgctggcaggcagcgccactttggtcgcccttggggcactggccttgtacgtcgcgaagccctccggctacgggaagcacacggagagcctgaagccggcggctacccgcctgccagcccgcgccgcctggttcctgcaggagctgccttccttcgcggtgcccgcggggatcctcgcccggcagcccctctccctcttcgggccacctgggacggtacttctgggcctcttctgcctacattacttccacaggacatttgtgtactcactgctcaatcgagggaggccttatccagctatactcattctcagaggcactgccttctgcactggaaatggagtccttcaaggctactatctgatttactgtgctgaataccctgatgggtggtacacagacatacggtttagcttgggtgtcttcttatttattttgggaatgggaataaacattcatagtgactatatattgcgccagctcaggaagcctggagaaatcagctacaggattccacaaggtggcttgtttacgtatgtttctggagccaatttcctcggtgagatcattgaatggatcggctatgccctggccacttggtccctcccagcacttgcatttgcatttttctcactttgtttccttgggctgcgagcttttcaccaccataggttctacctcaagatgtttgaggactaccccaaatctcggaaagcccttattccattcatcttttaaaggaaccaaattaaaaaggagcagagctcccacaatgctgatgaaaactgtcaagctgctgaaactgtaattttcatgatataatagtcccgtatatatgtaatagtaggtctcctggcgttctgccagctggcctggggattctgagtggtgtctgcttagagtttactcctacccttccagggacccctatcctgatccccaactgaagcttcaaaaagccacttttccaaatggcgacagttgcttcttagctattgctctgagaaagtacaaacttctcctatgtctttcaccgggcaatccaagtacatgtggcttcatacccactccctgtcaatgcaggacaactctgtaatcaagaattttttgacttgaaggcagtacttatagaccttattaaaggtatgcattttatacatgtaacagagtagcagaaatttaaactctgaagccacaaagacccagagcaaacccactcccaaatgaaaaccccagtcatggcttcctttttcttggttaattaggaaagatgagaaattattaggtagaccttgaatacaggagccctctcctcatagtgctgaaaagatactgatgcattgacctcatttcaaatttgtgcagtgtcttagttgatgagtgcctctgttttccagaagatttcacaatccccggaaaactggtatggctattcttgaaggccaggttttaataaccacaaacaaaaaggcatgaacctgggtggcttatgagagagtagagaacaacatgaccctggatggctactaagaggatagagaacagttttacaatagacattgcaaactctcatgtttttggaaactagtggcaatatccaaataatgagtagtgtaaaacaaagagaattaatgatgaggttacatgctgcttgcctccaccagatgtccacaacaatatgaagtacagcagaagccccaagcaactttcctttcctggagcttcttccttgtagttctcaggacctgttcaagaaggtgtctcctaggggcagcctgaatgcctccctcaaaggacctgcaggcagagactgaaaattgcagacagaggggcacgtctgggcagaaaacctgttttgtttggctcagacatatagttttttttttttttacaaagtttcaaaaacttaaaaatcaggagattccttcataaaactctagcattctagtttcatttaaaaagttggaggatctgaacatacagagcccacatttccacaccagaactggaactacgtagctagtaagcatttgagtttgcaaactcttgtgaaggggtcaccccagcatgagtgctgagatatggactctctaaggaaggggccgaacgcttgtaattggaatacatggaaatatttgtcttctcaggcctatgtttgcggaatgcattgtcaatatttagcaaactgttttgacaaatgagcaccagtggtactaagcacagaaactcactatataagtcacataggaaacttgaaaggtctgaggatgatgtagattactgaaaaatgcaaattgcaatcatataaataagtgtttttgttgttcattaaatacctttaaatcatg

SEQ ID NO: 673 - DNA, 8112 bp, Artificial Sequence
  NCBI Reference Sequence NM_001011645.2 669
gctgcgagcagagagggattcctcggaggtcatctgttccatcttcttgcctatgcaaatgcctgcctgaagctgctggaggctggctttgtaccggactttgtacagggaaccagggaaacgaatgcagagtgctcctgacattgcctgtcactttttcccatgatactctggcttcacagtttggagactgccagggaccatgttttgcccattgactattactttccaccccagaagacctgcctgatctgtggagatgaagcttctgggtgtcactatggagctctcacatgtggaagctgcaaggtcttcttcaaaagagccgctgaagggaaacagaagtacctgtgcgccagcagaaatgattgcactattgataaattccgaaggaaaaattgtccatcttgtcgtcttcggaaatgttatgaagcagggatgactctgggagcccggaagctgaagaaacttggtaatctgaaactacaggaggaaggagaggcttccagcaccaccagccccactgaggagacaacccagaagctgacagtgtcacacattgaaggctatgaatgtcagcccatctttctgaatgtcctggaagccattgagccaggtgtagtgtgtgctggacacgacaacaaccagcccgactcctttgcagccttgctctctagcctcaatgaactgggagagagacagcttgtacacgtggtcaagtgggccaaggccttgcctggcttccgcaacttacacgtggacgaccagatggctgtcattcagtactcctggatggggctcatggtgtttgccatgggctggcgatccttcaccaatgtcaactccaggatgctctacttcgcccctgatctggttttcaatgagtaccgcatgcacaagtcccggatgtacagccagtgtgtccgaatgaggcacctctctcaagagtttggatggctccaaatcaccccccaggaattcctgtgcatgaaagcactgctactcttcagcattattccagtggatgggctgaaaaatcaaaaattctttgatgaacttcgaatgaactacatcaaggaactcgatcgtatcattgcatgcaaaagaaaaaatcccacatcctgctcaagacgcttctaccagctcaccaagctcctggactccgtgcagcctattgcgagagagctgcatcagttcacttttgacctgctaatcaagtcacacatggtgagcgtggactttccggaaatgatggcagagatcatctctgtgcaagtgcccaagatcctttctgggaaagtcaagcccatctatttccacacccagtgaagcattggaaaccctatttccccaccccagctcatgccccctttcagatgtcttctgcctgttataactctgcactactcctctgcagtgccttggggaatttcctctattgatgtacagtctgtcatgaacatgttcctgaattctatttgctgggctttttttttctctttctctcctttctttttcttcttccctccctatctaaccctcccatggcaccttcagactttgcttcccattgtggctcctatctgtgttttgaatggtgttgtatgcctttaaatctgtgatgatcctcatatggcccagtgtcaagttgtgcttgtttacagcactactctgtgccagccacacaaacgtttacttatcttatgccacgggaagtttagagagctaagattatctggggaaatcaaaacaaaaacaagcaaacaaaaaaaaaaagcaaaaacaaaacaaaaaataagccaaaaaaccttgctagtgttttttcctcaaaaataaataaataaataaataaatacgtacatacatacacacatacatacaaacatatagaaatccccaaagaggccaatagtgacgagaaggtgaaaattgcaggcccatggggagttactgattttttcatctcctccctccacgggagactttattttctgccaatggctattgccattagagggcagagtgaccccagagctgagttgggcaggggggtggacagagaggagaggacaaggagggcaatggagcatcagtacctgcccacagccttggtccctgggggctagactgctcaactgtggagcaattcattatactgaaaatgtgcttgttgttgaaaatttgtctgcatgttaatgcctcacccccaaacccttttctctctcactctctgcctccaacttcagattgactttcaatagtttttctaagacctttgaactgaatgttctcttcagccaaaacttggcgacttccacagaaaagtctgaccactgagaagaaggagagcagagatttaaccctttgtaaggccccatttggatccaggtctgctttctcatgtgtgagtcagggaggagctggagccagaggagaagaaaatgatagcttggctgttctcctgcttaggacactgactgaatagttaaactctcactgccactaccttttccccacctttaaaagacctgaatgaagttttctgccaaactccgtgaagccacaagcaccttatgtcctcccttcagtgttttgtgggcctgaatttcatcacactgcatttcagccatggtcatcaagcctgtttgcttcttttgggcatgttcacagattctctgttaagagcccccaccaccaagaaggttagcaggccaacagctctgacatctatctgtagatgccagtagtcacaaagatttcttaccaactctcagatcgctggagcccttagacaaactggaaagaaggcatcaaagggatcaggcaagctgggcgtcttgcccttgtcccccagagatgataccctcccagcaagtggagaagttctcacttccttctttagagcagctaaaggggctacccagatcagggttgaagagaaaactcaattaccagggtgggaagaatgaaggcactagaaccagaaaccctgcaaatgctcttcttgtcacccagcatatccacctgcagaagtcatgagaagagagaaggaacaaagaggagactctgactactgaattaaaatcttcagcggcaaagcctaaagccagatggacaccatctggtgagtttactcatcatcctcctctgctgctgattctgggctctgacattgcccatactcactcagattccccacctttgttgctgcctcttagtcagagggaggccaaaccattgagactttctacagaaccatggcttctttcggaaaggtctggttggtgtggctccaatactttgccacccatgaactcagggtgtgccctgggacactggttttatatagtcttttggcacacctgtgttctgttgacttcgttcttcaagcccaagtgcaagggaaaatgtccacctactttctcatcttggcctctgcctccttacttagctcttaatctcatctgttgaactcaagaaatcaagggccagtcatcaagctgcccattttaattgattcactctgtttgttgagaggatagtttctgagtgacatgatatgatccacaagggtttccttccctgatttctgcattgatattaatagccaaacgaacttcaaaacagctttaaataacaagggagaggggaacctaagatgagtaatatgccaatccaagactgctggagaaaactaaagctgacaggttccctttttggggtgggatagacatgttctggttttctttattattacacaatctggctcatgtacaggatcacttttagctgttttaaacagaaaaaaatatccaccactcttttcagttacactaggttacattttaataggtcctttacatctgttttggaatgattttcatcttttgtgatacacagattgaattatatcattttcatatctctccttgtaaatactagaagctctcctttacatttctctatcaaatttttcatctttatgggtttcccaattgtgactcttgtcttcatgaatatatgtttttcatttgcaaaagccaaaaatcagtgaaacagcagtgtaattaaaagcaacaactggattactccaaatttccaaatgacaaaactagggaaaaatagcctacacaagcctttaggcctactctttctgtgcttgggtttgagtgaacaaaggagattttagcttggctctgttctcccatggatgaaaggaggaggattttttttttcttttggccattgatgttctagccaatgtaattgacagaagtctcattttgcatgcgctctgctctacaaacagagttggtatggttggtatactgtactcacctgtgagggactggccactcagacccacttagctggtgagctagaagatgaggatcactcactggaaaagtcacaaggaccatctccaaacaagttggcagtgctcgatgtggacgaagagtgaggaagagaaaaagaaggagcaccagggagaaggctccgtctgtgctgggcagcagacagctgccaggatcacgaactctgtagtcaaagaaaagagtcgtgtggcagtttcagctctcgttcattgggcagctcgcctaggcccagcctctgagctgacatgggagttgttggattctttgtttcatagctttttctatgccataggcaatattgttgttcttggaaagtttattatttttttaactcccttactctgagaaagggatattttgaaggactgtcatatatctttgaaaaaagaaaatctgtaatacatatatttttatgtatgttcactggcactaaaaaatatagagagcttcattctgtcctttgggtagttgctgaggtaattgtccaggttgaaaaataatgtgctgatgctagagtccctctctgtccatactctacttctaaatacatataggcatacatagcaagttttatttgacttgtactttaagagaaaatatgtccaccatccacatgatgcacaaatgagctaacattgagcttcaagtagcttctaagtgtttgtttcattaggcacagcacagatgtggcctttccccccttctctcccttgatatctggcagggcataaaggcccaggccacttcctctgccccttcccagccctgcaccaaagctgcatttcaggagactctctccagacagcccagtaactacccgagcatggcccctgcatagccctggaaaaataagaggctgactgtctacgaattatcttgtgccagttgcccaggtgagagggcactgggccaagggagtggttttcatgtttgacccactacaaggggtcatgggaatcaggaatgccaaagcaccagatcaaatccaaaacttaaagtcaaaataagccattcagcatgttcagtttcttggaaaaggaagtttctacccctgatgcctttgtaggcagatctgttctcaccattaatctttttgaaaatcttttaaagcagtttttaaaaagagagatgaaagcatcacattatataaccaaagattacattgtacctgctaagataccaaaattcataagggcagggggggagcaagcattagtgcctctttgataagctgtccaaagacagactaaaggactctgctggtgactgacttataagagctttgtgggtttttttttccctaataatatacatgtttagaagaattgaaaataatttcgggaaaatgggattatgggtccttcactaagtgattttataagcagaactggctttccttttctctagtagttgctgagcaaattgttgaagctccatcattgcatggttggaaatggagctgttcttagccactgtgtttgctagtgcccatgttagcttatctgaagatgtgaaacccttgctgataagggagcatttaaagtactagattttgcactagagggacagcaggcagaaatccttatttctgcccactttggatggcacaaaaagttatctgcagttgaaggcagaaagttgaaatacattgtaaatgaatatttgtatccatgtttcaaaattgaaatatatatatatatatatatatatatatatatatatatatagtgtgtgtgtgtgttctgatagctttaactttctctgcatctttatatttggttccagatcacacctgatgccatgtacttgtgagagaggatgcagttttgttttggaagctctctcagaacaaacaagacacctggattgatcagttaactaaaagttttctcccctattgggtttgacccacaggtcctgtgaaggagcagagggataaaaagagtagaggacatgatacattgtactttactagttcaagacagatgaatgtggaaagcataaaaactcaatggaactgactgagatttaccacagggaaggcccaaacttggggccaaaagcctacccaagtgattgaccagtggccccctaatgggacctgagctgttggaagaagagaactgttccttggtcttcaccatccttgtgagagaagggcagtttcctgcattggaacctggagcaagcgctctatctttcacacaaattccctcacctgagattgaggtgctcttgttactgggtgtctgtgtgctgtaattctggttttggatatgttctgtaaagattttgacaaatgaaaatgtgtttttctctgttaaaacttgtcagagtactagaagttgtatctctgtaggtgcaggtccatttctgcccacaggtagggtgtttttctttgattaagagattgacacttctgttgcctaggacctcccaactcaaccatttctaggtgaaggcagaaaaatccacattagttactcctcttcagacatttcagctgagataacaaatcttttggaattttttcacccatagaaagagtggtagatatttgaatttagcaggtggagtttcatagtaaaaacagcttttgactcagctttgatttatcctcatttgatttggccagaaagtaggtaatatgcattgattggcttctgattccaattcagtatagcaaggtgctaggttttttcctttccccacctgtctcttagcctggggaattaaatgagaagccttagaatgggtggcccttgtgacctgaaacacttcccacataagctacttaacaagattgtcatggagctgcagattccattgcccaccaaagactagaacacacacatatccatacaccaaaggaaagacaattctgaaatgctgtttctctggtggttccctctctggctgctgcctcacagtatgggaacctgtactctgcagaggtgacaggccagatttgcattatctcacaaccttagcccttggtgctaactgtcctacagtgaagtgcctggggggttgtcctatcccataagccacttggatgctgacagcagccaccatcagaatgacccacgcaaaaaaaagaaaaaaaaaattaaaaagtcccctcacaacccagtgacacctttctgctttcctctagactggaacattgattagggagtgcctcagacatgacattcttgtgctgtccttggaattaatctggcagcaggagggagcagactatgtaaacagagataaaaattaattttcaatattgaaggaaaaaagaaataagaagagagagagaaagaaagcatcacacaaagattttcttaaaagaaacaattttgcttgaaatctctttagatggggctcatttctcacggtggcacttggcctccactgggcagcaggaccagctccaagcgctagtgttctgttctctttttgtaatcttggaatcttttgttgctctaaatacaattaaaaatggcagaaacttgtttgttggactacatgtgtgactttgggtctgtctctgcctctgctttcagaaatgtcatccattgtgtaaaatattggcttactggtctgccagctaaaacttggccacatcccctgttatggctgcaggatcgagttattgttaacaaagagacccaagaaaagctgctaatgtcctcttatcattgttgttaatttgttaaaacataaagaaatctaaaatttcaaaaaa